European Patent Application EP 4 144 844 A1, published March 8, 2023. Title: PROTECTED DNA TEMPLATES FOR GENE MODIFICATION AND INCREASED HOMOLOGOUS RECOMBINATION IN CELLS AND METHODS OF USE. Applicant: DuPont US Holding, LLC. Application EP. The sequence listing filed with the application follows.

SEQUENCE LISTING (72 sequences)

SEQ ID NO: 1 - protein, 1372 aa, Streptococcus pyogenes
MDKKYSIGLDIGTNSVGWAVITDEYKVPSKKFKVLGNTDRHSIKKNLIGALLFDSGETAEATRLKRTARRRYTRRKNRICYLQEIFSNEMAKVDDSFFHRLEESFLVEEDKKHERHPIFGNIVDEVAYHEKYPTIYHLRKKLVDSTDKADLRLIYLALAHMIKFRGHFLIEGDLNPDNSDVDKLFIQLVQTYNQLFEENPINASGVDAKAILSARLSKSRRLENLIAQLPGEKKNGLFGNLIALSLGLTPNFKSNFDLAEDAKLQLSKDTYDDDLDNLLAQIGDQYADLFLAAKNLSDAILLSDILRVNTEITKAPLSASMIKRYDEHHQDLTLLKALVRQQLPEKYKEIFFDQSKNGYAGYIDGGASQEEFYKFIKPILEKMDGTEELLVKLNREDLLRKQRTFDNGSIPHQIHLGELHAILRRQEDFYPFLKDNREKIEKILTFRIPYYVGPLARGNSRFAWMTRKSEETITPWNFEEVVDKGASAQSFIERMTNFDKNLPNEKVLPKHSLLYEYFTVYNELTKVKYVTEGMRKPAFLSGEQKKAIVDLLFKTNRKVTVKQLKEDYFKKIECFDSVEISGVEDRFNASLGTYHDLLKIIKDKDFLDNEENEDILEDIVLTLTLFEDREMIEERLKTYAHLFDDKVMKQLKRRRYTGWGRLSRKLINGIRDKQSGKTILDFLKSDGFANRNFMQLIHDDSLTFKEDIQKAQVSGQGDSLHEHIANLAGSPAIKKGILQTVKVVDELVKVMGRHKPENIVIEMARENQTTQKGQKNSRERMKRIEEGIKELGSQILKEHPVENTQLQNEKLYLYYLQNGRDMYVDQELDINRLSDYDVDHIVPQSFLKDDSIDNKVLTRSDKNRGKSDNVPSEEVVKKMKNYWRQLLNAKLITQRKFDNLTKAERGGLSELDKAGFIKRQLVETRQITKHVAQILDSRMNTKYDENDKLIREVKVITLKSKLVSDFRKDFQFYKVREINNYHHAHDAYLNAVVGTALIKKYPKLESEFVYGDYKVYDVRKMIAKSEQEIGKATAKYFFYSNIMNFFKTEITLANGEIRKRPLIETNGETGEIVWDKGRDFATVRKVLSMPQVNIVKKTEVQTGGFSKESILPKRNSDKLIARKKDWDPKKYGGFDSPTVAYSVLVVAKVEKGKSKKLKSVKELLGITIMERSSFEKNPIDFLEAKGYKEVKKDLIIKLPKYSLFELENGRKRMLASAGELQKGNELALPSKYVNFLYLASHYEKLKGSPEDNEQKQLFVEQHKHYLDEIIEQISEFSKRVILADANLDKVLSAYNKHRDKPIREQAENIIHLFTLTNLGAPAAFKYFDTTIDRKRYTSTKEVLDATLIHQSITGLYETRIDLSQLGGDSRAD

SEQ ID NO: 2 - DNA, 4140 bp, synthetic construct
  misc_feature 1..4140: note = Yarrowia codon optimized Cas9
  source 1..4140: mol_type = other DNA
atggacaagaaatactccatcggcctggacattggaaccaactctgtcggctgggctgtcatcaccgacgagtacaaggtgccctccaagaaattcaaggtcctcggaaacaccgatcgacactccatcaagaaaaacctcattggtgccctgttgttcgattctggcgagactgccgaagctaccagactcaagcgaactgctcggcgacgttacacccgacggaagaaccgaatctgctacctgcaggagatcttttccaacgagatggccaaggtggacgattcgttctttcatcgactggaggaatccttcctcgtcgaggaagacaagaaacacgagcgtcatcccatctttggcaacattgtggacgaggttgcttaccacgagaagtatcctaccatctaccatctccgaaagaaactcgtcgattccaccgacaaggcggatctcagacttatctacctcgctctggcacacatgatcaagtttcgaggtcatttcctcatcgagggcgatctcaatcccgacaacagcgatgtggacaagctgttcattcagctcgttcagacctacaaccagctgttcgaggaaaaccccatcaatgcctccggagtcgatgcaaaggccatcttgtctgctcgactctcgaagagcagacgactggagaacctcattgcccaacttcctggcgagaaaaagaacggactgtttggcaacctcattgccctttctcttggtctcacacccaacttcaagtccaacttcgatctggcggaggacgccaagctccagctgtccaaggacacctacgacgatgacctcgacaacctgcttgcacagattggcgatcagtacgccgacctgtttctcgctgccaagaacctttcggatgctattctcttgtctgacattctgcgagtcaacaccgagatcacaaaggctcccctttctgcctccatgatcaagcgatacgacgagcaccatcaggatctcacactgctcaaggctcttgtccgacagcaactgcccgagaagtacaaggagatctttttcgatcagtcgaagaacggctacgctggatacatcgacggcggagcctctcaggaagagttctacaagttcatcaagccaattctcgagaagatggacggaaccgaggaactgcttgtcaagctcaatcgagaggatctgcttcggaagcaacgaaccttcgacaacggcagcattcctcatcagatccacctcggtgagctgcacgccattcttcgacgtcaggaagacttctacccctttctcaaggacaaccgagagaagatcgagaagattcttacctttcgaatcccctactatgttggtcctcttgccagaggaaactctcgatttgcttggatgactcgaaagtccgaggaaaccatcactccctggaacttcgaggaagtcgtggacaagggtgcctctgcacagtccttcatcgagcgaatgaccaacttcgacaagaatctgcccaacgagaaggttcttcccaagcattcgctgctctacgagtactttacagtctacaacgaactcaccaaagtcaagtacgttaccgagggaatgcgaaagcctgccttcttgtctggcgaacagaagaaagccattgtcgatctcctgttcaagaccaaccgaaaggtcactgttaagcagctcaaggaggactacttcaagaaaatcgagtgtttcgacagcgtcgagatttccggagttgaggaccgattcaacgcctctttgggcacctatcacgatctgctcaagattatcaaggacaaggattttctcgacaacgaggaaaacgaggacattctggaggacatcgtgctcactcttaccctgttcgaagatcgggagatgatcgaggaacgactcaagacatacgctcacctgttcgacgacaaggtcatgaaacaactcaagcgacgtagatacaccggctggggaagactttcgcgaaagctcatcaacggcatcagagacaagcagtccggaaagaccattctggactttctcaagtccgatggctttgccaaccgaaacttcatgcagctcattcacgacgattctcttaccttcaaggaggacatccagaaggcacaagtgtccggtcagggcgacagcttgcacgaacatattgccaacctggctggttcgccagccatcaagaaaggcattctccagactgtcaaggttgtcgacgagctggtgaaggtcatgggacgtcacaagcccgagaacattgtgatcgagatggccagagagaaccagacaactcaaaagggtcagaaaaactcgcgagagcggatgaagcgaatcgaggaaggcatcaaggagctgggatcccagattctcaaggagcatcccgtcgagaacactcaactgcagaacgagaagctgtatctctactatctgcagaatggtcgagacatgtacgtggatcaggaactggacatcaatcgtctcagcgactacgatgtggaccacattgtccctcaatcctttctcaaggacgattctatcgacaacaaggtccttacacgatccgacaagaacagaggcaagtcggacaacgttcccagcgaagaggtggtcaaaaagatgaagaactactggcgacagctgctcaacgccaagctcattacccagcgaaagttcgacaatcttaccaaggccgagcgaggcggtctgtccgagctcgacaaggctggcttcatcaagcgtcaactcgtcgagaccagacagatcacaaagcacgtcgcacagattctcgattctcggatgaacaccaagtacgacgagaacgacaagctcatccgagaggtcaaggtgattactctcaagtccaaactggtctccgatttccgaaaggactttcagttctacaaggtgcgagagatcaacaattaccaccatgcccacgatgcttacctcaacgccgtcgttggcactgcgctcatcaagaaataccccaagctcgaaagcgagttcgtttacggcgattacaaggtctacgacgttcgaaagatgattgccaagtccgaacaggagattggcaaggctactgccaagtacttcttttactccaacatcatgaactttttcaagaccgagatcaccttggccaacggagagattcgaaagagaccacttatcgagaccaacggcgaaactggagagatcgtgtgggacaagggtcgagactttgcaaccgtgcgaaaggttctgtcgatgcctcaggtcaacatcgtcaagaaaaccgaggttcagactggcggattctccaaggagtcgattctgcccaagcgaaactccgacaagctcatcgctcgaaagaaagactgggatcccaagaaatacggtggcttcgattctcctaccgtcgcctattccgtgcttgtcgttgcgaaggtcgagaagggcaagtccaaaaagctcaagtccgtcaaggagctgctcggaattaccatcatggagcgatcgagcttcgagaagaatcccatcgacttcttggaagccaagggttacaaggaggtcaagaaagacctcattatcaagctgcccaagtactctctgttcgaactggagaacggtcgaaagcgtatgctcgcctccgctggcgagctgcagaagggaaacgagcttgccttgccttcgaagtacgtcaactttctctatctggcttctcactacgagaagctcaagggttctcccgaggacaacgaacagaagcaactcttcgttgagcagcacaaacattacctcgacgagattatcgagcagatttccgagttttcgaagcgagtcatcctggctgatgccaacttggacaaggtgctctctgcctacaacaagcatcgggacaaacccattcgagaacaggcggagaacatcattcacctgtttactcttaccaacctgggtgctcctgcagctttcaagtacttcgataccactatcgaccgaaagcggtacacatccaccaaggaggttctcgatgccaccctgattcaccagtccatcactggcctgtacgagacccgaatcgacctgtctcagcttggtggcgactccagagccgatcccaagaaaaagcgaaaggtctaa

SEQ ID NO: 3 - protein, 7 aa, SV40
PKKKRKV

SEQ ID NO: 4 - DNA, 543 bp, YArrowia lipolytica
  source 1..543: mol_type = genomic DNA
tcgacgtttaaaccatcatctaagggcctcaaaactacctcggaactgctgcgctgatctggacaccacagaggttccgagcactttaggttgcaccaaatgtcccaccaggtgcaggcagaaaacgctggaacagcgtgtacagtttgtcttaacaaaaagtgagggcgctgaggtcgagcagggtggtgtgacttgttatagcctttagagctgcgaaagcgcgtatggatttggctcatcaggccagattgagggtctgtggacacatgtcatgttagtgtacttcaatcgccccctggatatagccccgacaataggccgtggcctcatttttttgccttccgcacatttccattgctcggtacccacaccttgcttctcctgcacttgccaaccttaatactggtttacattgaccaacatcttacaagcggggggcttgtctagggtatatataaacagtggctctcccaatcggttgccagtctcttttttcctttctttccccacagattcgaaatctaaactacacatcacacc

SEQ ID NO: 5 - DNA, 4683 bp, synthetic construct
  misc_feature 1..4683: note = Yarrowia optimized expression cassette
  source 1..4683: mol_type = other DNA
tcgacgtttaaaccatcatctaagggcctcaaaactacctcggaactgctgcgctgatctggacaccacagaggttccgagcactttaggttgcaccaaatgtcccaccaggtgcaggcagaaaacgctggaacagcgtgtacagtttgtcttaacaaaaagtgagggcgctgaggtcgagcagggtggtgtgacttgttatagcctttagagctgcgaaagcgcgtatggatttggctcatcaggccagattgagggtctgtggacacatgtcatgttagtgtacttcaatcgccccctggatatagccccgacaataggccgtggcctcatttttttgccttccgcacatttccattgctcggtacccacaccttgcttctcctgcacttgccaaccttaatactggtttacattgaccaacatcttacaagcggggggcttgtctagggtatatataaacagtggctctcccaatcggttgccagtctcttttttcctttctttccccacagattcgaaatctaaactacacatcacaccatggacaagaaatactccatcggcctggacattggaaccaactctgtcggctgggctgtcatcaccgacgagtacaaggtgccctccaagaaattcaaggtcctcggaaacaccgatcgacactccatcaagaaaaacctcattggtgccctgttgttcgattctggcgagactgccgaagctaccagactcaagcgaactgctcggcgacgttacacccgacggaagaaccgaatctgctacctgcaggagatcttttccaacgagatggccaaggtggacgattcgttctttcatcgactggaggaatccttcctcgtcgaggaagacaagaaacacgagcgtcatcccatctttggcaacattgtggacgaggttgcttaccacgagaagtatcctaccatctaccacctgcgaaagaaactcgtcgattccaccgacaaggcggatctcagacttatctacctcgctctggcacacatgatcaagtttcgaggtcatttcctcatcgagggcgatctcaatcccgacaacagcgatgtggacaagctgttcattcagctcgttcagacctacaaccagctgttcgaggaaaaccccatcaatgcctccggagtcgatgcaaaggccatcttgtctgctcgactctcgaagagcagacgactggagaacctcattgcccaacttcctggcgagaaaaagaacggactgtttggcaacctcattgccctttctcttggtctcacacccaacttcaagtccaacttcgatctggcggaggacgccaagctccagctgtccaaggacacctacgacgatgacctcgacaacctgcttgcacagattggcgatcagtacgccgacctgtttctcgctgccaagaacctttcggatgctattctcttgtctgacattctgcgagtcaacaccgagatcacaaaggctcccctttctgcctccatgatcaagcgatacgacgagcaccatcaggatctcacactgctcaaggctcttgtccgacagcaactgcccgagaagtacaaggagatctttttcgatcagtcgaagaacggctacgctggatacatcgacggcggagcctctcaggaagagttctacaagttcatcaagccaattctcgagaagatggacggaaccgaggaactgcttgtcaagctcaatcgagaggatctgcttcggaagcaacgaaccttcgacaacggcagcattcctcatcagatccacctcggtgagctgcacgccattcttcgacgtcaggaagacttctacccctttctcaaggacaaccgagagaagatcgagaagattcttacctttcgaatcccctactatgttggtcctcttgccagaggaaactctcgatttgcttggatgactcgaaagtccgaggaaaccatcactccctggaacttcgaggaagtcgtggacaagggtgcctctgcacagtccttcatcgagcgaatgaccaacttcgacaagaatctgcccaacgagaaggttcttcccaagcattcgctgctctacgagtactttacagtctacaacgaactcaccaaagtcaagtacgttaccgagggaatgcgaaagcctgccttcttgtctggcgaacagaagaaagccattgtcgatctcctgttcaagaccaaccgaaaggtcactgttaagcagctcaaggaggactacttcaagaaaatcgagtgtttcgacagcgtcgagatttccggagttgaggaccgattcaacgcctctttgggcacctatcacgatctgctcaagattatcaaggacaaggattttctcgacaacgaggaaaacgaggacattctggaggacatcgtgctcactcttaccctgttcgaagatcgggagatgatcgaggaacgactcaagacatacgctcacctgttcgacgacaaggtcatgaaacaactcaagcgacgtagatacaccggctggggaagactttcgcgaaagctcatcaacggcatcagagacaagcagtccggaaagaccattctggactttctcaagtccgatggctttgccaaccgaaacttcatgcagctcattcacgacgattctcttaccttcaaggaggacatccagaaggcacaagtgtccggtcagggcgacagcttgcacgaacatattgccaacctggctggttcgccagccatcaagaaaggcattctccagactgtcaaggttgtcgacgagctggtgaaggtcatgggacgtcacaagcccgagaacattgtgatcgagatggccagagagaaccagacaactcaaaagggtcagaaaaactcgcgagagcggatgaagcgaatcgaggaaggcatcaaggagctgggatcccagattctcaaggagcatcccgtcgagaacactcaactgcagaacgagaagctgtatctctactatctgcagaatggtcgagacatgtacgtggatcaggaactggacatcaatcgtctcagcgactacgatgtggaccacattgtccctcaatcctttctcaaggacgattctatcgacaacaaggtccttacacgatccgacaagaacagaggcaagtcggacaacgttcccagcgaagaggtggtcaaaaagatgaagaactactggcgacagctgctcaacgccaagctcattacccagcgaaagttcgacaatcttaccaaggccgagcgaggcggtctgtccgagctcgacaaggctggcttcatcaagcgtcaactcgtcgagaccagacagatcacaaagcacgtcgcacagattctcgattctcggatgaacaccaagtacgacgagaacgacaagctcatccgagaggtcaaggtgattactctcaagtccaaactggtctccgatttccgaaaggactttcagttctacaaggtgcgagagatcaacaattaccaccatgcccacgatgcttacctcaacgccgtcgttggcactgcgctcatcaagaaataccccaagctcgaaagcgagttcgtttacggcgattacaaggtctacgacgttcgaaagatgattgccaagtccgaacaggagattggcaaggctactgccaagtacttcttttactccaacatcatgaactttttcaagaccgagatcaccttggccaacggagagattcgaaagagaccacttatcgagaccaacggcgaaactggagagatcgtgtgggacaagggtcgagactttgcaaccgtgcgaaaggttctgtcgatgcctcaggtcaacatcgtcaagaaaaccgaggttcagactggcggattctccaaggagtcgattctgcccaagcgaaactccgacaagctcatcgctcgaaagaaagactgggatcccaagaaatacggtggcttcgattctcctaccgtcgcctattccgtgcttgtcgttgcgaaggtcgagaagggcaagtccaaaaagctcaagtccgtcaaggagctgctcggaattaccatcatggagcgatcgagcttcgagaagaatcccatcgacttcttggaagccaagggttacaaggaggtcaagaaagacctcattatcaagctgcccaagtactctctgttcgaactggagaacggtcgaaagcgtatgctcgcctccgctggcgagctgcagaagggaaacgagcttgccttgccttcgaagtacgtcaactttctctatctggcttctcactacgagaagctcaagggttctcccgaggacaacgaacagaagcaactcttcgttgagcagcacaaacattacctcgacgagattatcgagcagatttccgagttttcgaagcgagtcatcctggctgatgccaacttggacaaggtgctctctgcctacaacaagcatcgggacaaacccattcgagaacaggcggagaacatcattcacctgtttactcttaccaacctgggtgctcctgcagctttcaagtacttcgataccactatcgaccgaaagcggtacacatccaccaaggaggttctcgatgccaccctgattcaccagtccatcactggcctgtacgagacccgaatcgacctgtctcagcttggtggcgactccagagccgatcccaagaaaaagcgaaaggtctaa

SEQ ID NO: 6 - DNA, 10706 bp, synthetic construct
  misc_feature 1..10706: note = pZufCas9
  source 1..10706: mol_type = other DNA
catggacaagaaatactccatcggcctggacattggaaccaactctgtcggctgggctgtcatcaccgacgagtacaaggtgccctccaagaaattcaaggtcctcggaaacaccgatcgacactccatcaagaaaaacctcattggtgccctgttgttcgattctggcgagactgccgaagctaccagactcaagcgaactgctcggcgacgttacacccgacggaagaaccgaatctgctacctgcaggagatcttttccaacgagatggccaaggtggacgattcgttctttcatcgactggaggaatccttcctcgtcgaggaagacaagaaacacgagcgtcatcccatctttggcaacattgtggacgaggttgcttaccacgagaagtatcctaccatctaccacctgcgaaagaaactcgtcgattccaccgacaaggcggatctcagacttatctacctcgctctggcacacatgatcaagtttcgaggtcatttcctcatcgagggcgatctcaatcccgacaacagcgatgtggacaagctgttcattcagctcgttcagacctacaaccagctgttcgaggaaaaccccatcaatgcctccggagtcgatgcaaaggccatcttgtctgctcgactctcgaagagcagacgactggagaacctcattgcccaacttcctggcgagaaaaagaacggactgtttggcaacctcattgccctttctcttggtctcacacccaacttcaagtccaacttcgatctggcggaggacgccaagctccagctgtccaaggacacctacgacgatgacctcgacaacctgcttgcacagattggcgatcagtacgccgacctgtttctcgctgccaagaacctttcggatgctattctcttgtctgacattctgcgagtcaacaccgagatcacaaaggctcccctttctgcctccatgatcaagcgatacgacgagcaccatcaggatctcacactgctcaaggctcttgtccgacagcaactgcccgagaagtacaaggagatctttttcgatcagtcgaagaacggctacgctggatacatcgacggcggagcctctcaggaagagttctacaagttcatcaagccaattctcgagaagatggacggaaccgaggaactgcttgtcaagctcaatcgagaggatctgcttcggaagcaacgaaccttcgacaacggcagcattcctcatcagatccacctcggtgagctgcacgccattcttcgacgtcaggaagacttctacccctttctcaaggacaaccgagagaagatcgagaagattcttacctttcgaatcccctactatgttggtcctcttgccagaggaaactctcgatttgcttggatgactcgaaagtccgaggaaaccatcactccctggaacttcgaggaagtcgtggacaagggtgcctctgcacagtccttcatcgagcgaatgaccaacttcgacaagaatctgcccaacgagaaggttcttcccaagcattcgctgctctacgagtactttacagtctacaacgaactcaccaaagtcaagtacgttaccgagggaatgcgaaagcctgccttcttgtctggcgaacagaagaaagccattgtcgatctcctgttcaagaccaaccgaaaggtcactgttaagcagctcaaggaggactacttcaagaaaatcgagtgtttcgacagcgtcgagatttccggagttgaggaccgattcaacgcctctttgggcacctatcacgatctgctcaagattatcaaggacaaggattttctcgacaacgaggaaaacgaggacattctggaggacatcgtgctcactcttaccctgttcgaagatcgggagatgatcgaggaacgactcaagacatacgctcacctgttcgacgacaaggtcatgaaacaactcaagcgacgtagatacaccggctggggaagactttcgcgaaagctcatcaacggcatcagagacaagcagtccggaaagaccattctggactttctcaagtccgatggctttgccaaccgaaacttcatgcagctcattcacgacgattctcttaccttcaaggaggacatccagaaggcacaagtgtccggtcagggcgacagcttgcacgaacatattgccaacctggctggttcgccagccatcaagaaaggcattctccagactgtcaaggttgtcgacgagctggtgaaggtcatgggacgtcacaagcccgagaacattgtgatcgagatggccagagagaaccagacaactcaaaagggtcagaaaaactcgcgagagcggatgaagcgaatcgaggaaggcatcaaggagctgggatcccagattctcaaggagcatcccgtcgagaacactcaactgcagaacgagaagctgtatctctactatctgcagaatggtcgagacatgtacgtggatcaggaactggacatcaatcgtctcagcgactacgatgtggaccacattgtccctcaatcctttctcaaggacgattctatcgacaacaaggtccttacacgatccgacaagaacagaggcaagtcggacaacgttcccagcgaagaggtggtcaaaaagatgaagaactactggcgacagctgctcaacgccaagctcattacccagcgaaagttcgacaatcttaccaaggccgagcgaggcggtctgtccgagctcgacaaggctggcttcatcaagcgtcaactcgtcgagaccagacagatcacaaagcacgtcgcacagattctcgattctcggatgaacaccaagtacgacgagaacgacaagctcatccgagaggtcaaggtgattactctcaagtccaaactggtctccgatttccgaaaggactttcagttctacaaggtgcgagagatcaacaattaccaccatgcccacgatgcttacctcaacgccgtcgttggcactgcgctcatcaagaaataccccaagctcgaaagcgagttcgtttacggcgattacaaggtctacgacgttcgaaagatgattgccaagtccgaacaggagattggcaaggctactgccaagtacttcttttactccaacatcatgaactttttcaagaccgagatcaccttggccaacggagagattcgaaagagaccacttatcgagaccaacggcgaaactggagagatcgtgtgggacaagggtcgagactttgcaaccgtgcgaaaggttctgtcgatgcctcaggtcaacatcgtcaagaaaaccgaggttcagactggcggattctccaaggagtcgattctgcccaagcgaaactccgacaagctcatcgctcgaaagaaagactgggatcccaagaaatacggtggcttcgattctcctaccgtcgcctattccgtgcttgtcgttgcgaaggtcgagaagggcaagtccaaaaagctcaagtccgtcaaggagctgctcggaattaccatcatggagcgatcgagcttcgagaagaatcccatcgacttcttggaagccaagggttacaaggaggtcaagaaagacctcattatcaagctgcccaagtactctctgttcgaactggagaacggtcgaaagcgtatgctcgcctccgctggcgagctgcagaagggaaacgagcttgccttgccttcgaagtacgtcaactttctctatctggcttctcactacgagaagctcaagggttctcccgaggacaacgaacagaagcaactcttcgttgagcagcacaaacattacctcgacgagattatcgagcagatttccgagttttcgaagcgagtcatcctggctgatgccaacttggacaaggtgctctctgcctacaacaagcatcgggacaaacccattcgagaacaggcggagaacatcattcacctgtttactcttaccaacctgggtgctcctgcagctttcaagtacttcgataccactatcgaccgaaagcggtacacatccaccaaggaggttctcgatgccaccctgattcaccagtccatcactggcctgtacgagacccgaatcgacctgtctcagcttggtggcgactccagagccgatcccaagaaaaagcgaaaggtctaagcggccgcaagtgtggatggggaagtgagtgcccggttctgtgtgcacaattggcaatccaagatggatggattcaacacagggatatagcgagctacgtggtggtgcgaggatatagcaacggatatttatgtttgacacttgagaatgtacgatacaagcactgtccaagtacaatactaaacatactgtacatactcatactcgtacccgggcaacggtttcacttgagtgcagtggctagtgctcttactcgtacagtgtgcaatactgcgtatcatagtctttgatgtatatcgtattcattcatgttagttgcgtacgagccggaagcataaagtgtaaagcctggggtgcctaatgagtgagctaactcacattaattgcgttgcgctcactgcccgctttccagtcgggaaacctgtcgtgccagctgcattaatgaatcggccaacgcgcggggagaggcggtttgcgtattgggcgctcttccgcttcctcgctcactgactcgctgcgctcggtcgttcggctgcggcgagcggtatcagctcactcaaaggcggtaatacggttatccacagaatcaggggataacgcaggaaagaacatgtgagcaaaaggccagcaaaaggccaggaaccgtaaaaaggccgcgttgctggcgtttttccataggctccgcccccctgacgagcatcacaaaaatcgacgctcaagtcagaggtggcgaaacccgacaggactataaagataccaggcgtttccccctggaagctccctcgtgcgctctcctgttccgaccctgccgcttaccggatacctgtccgcctttctcccttcgggaagcgtggcgctttctcatagctcacgctgtaggtatctcagttcggtgtaggtcgttcgctccaagctgggctgtgtgcacgaaccccccgttcagcccgaccgctgcgccttatccggtaactatcgtcttgagtccaacccggtaagacacgacttatcgccactggcagcagccactggtaacaggattagcagagcgaggtatgtaggcggtgctacagagttcttgaagtggtggcctaactacggctacactagaaggacagtatttggtatctgcgctctgctgaagccagttaccttcggaaaaagagttggtagctcttgatccggcaaacaaaccaccgctggtagcggtggtttttttgtttgcaagcagcagattacgcgcagaaaaaaaggatctcaagaagatcctttgatcttttctacggggtctgacgctcagtggaacgaaaactcacgttaagggattttggtcatgagattatcaaaaaggatcttcacctagatccttttaaattaaaaatgaagttttaaatcaatctaaagtatatatgagtaaacttggtctgacagttaccaatgcttaatcagtgaggcacctatctcagcgatctgtctatttcgttcatccatagttgcctgactccccgtcgtgtagataactacgatacgggagggcttaccatctggccccagtgctgcaatgataccgcgagacccacgctcaccggctccagatttatcagcaataaaccagccagccggaagggccgagcgcagaagtggtcctgcaactttatccgcctccatccagtctattaattgttgccgggaagctagagtaagtagttcgccagttaatagtttgcgcaacgttgttgccattgctacaggcatcgtggtgtcacgctcgtcgtttggtatggcttcattcagctccggttcccaacgatcaaggcgagttacatgatcccccatgttgtgcaaaaaagcggttagctccttcggtcctccgatcgttgtcagaagtaagttggccgcagtgttatcactcatggttatggcagcactgcataattctcttactgtcatgccatccgtaagatgcttttctgtgactggtgagtactcaaccaagtcattctgagaatagtgtatgcggcgaccgagttgctcttgcccggcgtcaatacgggataataccgcgccacatagcagaactttaaaagtgctcatcattggaaaacgttcttcggggcgaaaactctcaaggatcttaccgctgttgagatccagttcgatgtaacccactcgtgcacccaactgatcttcagcatcttttactttcaccagcgtttctgggtgagcaaaaacaggaaggcaaaatgccgcaaaaaagggaataagggcgacacggaaatgttgaatactcatactcttcctttttcaatattattgaagcatttatcagggttattgtctcatgagcggatacatatttgaatgtatttagaaaaataaacaaataggggttccgcgcacatttccccgaaaagtgccacctgacgcgccctgtagcggcgcattaagcgcggcgggtgtggtggttacgcgcagcgtgaccgctacacttgccagcgccctagcgcccgctcctttcgctttcttcccttcctttctcgccacgttcgccggctttccccgtcaagctctaaatcgggggctccctttagggttccgatttagtgctttacggcacctcgaccccaaaaaacttgattagggtgatggttcacgtagtgggccatcgccctgatagacggtttttcgccctttgacgttggagtccacgttctttaatagtggactcttgttccaaactggaacaacactcaaccctatctcggtctattcttttgatttataagggattttgccgatttcggcctattggttaaaaaatgagctgatttaacaaaaatttaacgcgaattttaacaaaatattaacgcttacaatttccattcgccattcaggctgcgcaactgttgggaagggcgatcggtgcgggcctcttcgctattacgccagctggcgaaagggggatgtgctgcaaggcgattaagttgggtaacgccagggttttcccagtcacgacgttgtaaaacgacggccagtgaattgtaatacgactcactatagggcgaattgggtaccgggccccccctcgaggtcgatggtgtcgataagcttgatatcgaattcatgtcacacaaaccgatcttcgcctcaaggaaacctaattctacatccgagagactgccgagatccagtctacactgattaattttcgggccaataatttaaaaaaatcgtgttatataatattatatgtattatatatatacatcatgatgatactgacagtcatgtcccattgctaaatagacagactccatctgccgcctccaactgatgttctcaatatttaaggggtcatctcgcattgtttaataataaacagactccatctaccgcctccaaatgatgttctcaaaatatattgtatgaacttatttttattacttagtattattagacaacttacttgctttatgaaaaacacttcctatttaggaaacaatttataatggcagttcgttcatttaacaatttatgtagaataaatgttataaatgcgtatgggaaatcttaaatatggatagcataaatgatatctgcattgcctaattcgaaatcaacagcaacgaaaaaaatcccttgtacaacataaatagtcatcgagaaatatcaactatcaaagaacagctattcacacgttactattgagattattattggacgagaatcacacactcaactgtctttctctcttctagaaatacaggtacaagtatgtactattctcattgttcatacttctagtcatttcatcccacatattccttggatttctctccaatgaatgacattctatcttgcaaattcaacaattataataagatataccaaagtagcggtatagtggcaatcaaaaagcttctctggtgtgcttctcgtatttatttttattctaatgatccattaaaggtatatatttatttcttgttatataatccttttgtttattacatgggctggatacataaaggtattttgatttaattttttgcttaaattcaatcccccctcgttcagtgtcaactgtaatggtaggaaattaccatacttttgaagaagcaaaaaaaatgaaagaaaaaaaaaatcgtatttccaggttagacgttccgcagaatctagaatgcggtatgcggtacattgttcttcgaacgtaaaagttgcgctccctgagatattgtacatttttgcttttacaagtacaagtacatcgtacaactatgtactactgttgatgcatccacaacagtttgttttgtttttttttgttttttttttttctaatgattcattaccgctatgtatacctacttgtacttgtagtaagccgggttattggcgttcaattaatcatagacttatgaatctgcacggtgtgcgctgcgagttacttttagcttatgcatgctacttgggtgtaatattgggatctgttcggaaatcaacggatgctcaatcgatttcgacagtaattaattaagtcatacacaagtcagctttcttcgagcctcatataagtataagtagttcaacgtattagcactgtacccagcatctccgtatcgagaaacacaacaacatgccccattggacagatcatgcggatacacaggttgtgcagtatcatacatactcgatcagacaggtcgtctgaccatcatacaagctgaacaagcgctccatacttgcacgctctctatatacacagttaaattacatatccatagtctaacctctaacagttaatcttctggtaagcctcccagccagccttctggtatcgcttggcctcctcaataggatctcggttctggccgtacagacctcggccgacaattatgatatccgttccggtagacatgacatcctcaacagttcggtactgctgtccgagagcgtctcccttgtcgtcaagacccaccccgggggtcagaataagccagtcctcagagtcgcccttaggtcggttctgggcaatgaagccaaccacaaactcggggtcggatcgggcaagctcaatggtctgcttggagtactcgccagtggccagagagcccttgcaagacagctcggccagcatgagcagacctctggccagcttctcgttgggagaggggactaggaactccttgtactgggagttctcgtagtcagagacgtcctccttcttctgttcagagacagtttcctcggcaccagctcgcaggccagcaatgattccggttccgggtacaccgtgggcgttggtgatatcggaccactcggcgattcggtgacaccggtactggtgcttgacagtgttgccaatatctgcgaactttctgtcctcgaacaggaagaaaccgtgcttaagagcaagttccttgagggggagcacagtgccggcgtaggtgaagtcgtcaatgatgtcgatatgggttttgatcatgcacacataaggtccgaccttatcggcaagctcaatgagctccttggtggtggtaacatccagagaagcacacaggttggttttcttggctgccacgagcttgagcactcgagcggcaaaggcggacttgtggacgttagctcgagcttcgtaggagggcattttggtggtgaagaggagactgaaataaatttagtctgcagaactttttatcggaaccttatctggggcagtgaagtatatgttatggtaatagttacgagttagttgaacttatagatagactggactatacggctatcggtccaaattagaaagaacgtcaatggctctctgggcgtcgcctttgccgacaaaaatgtgatcatgatgaaagccagcaatgacgttgcagctgatattgttgtcggccaaccgcgccgaaaacgcagctgtcagacccacagcctccaacgaagaatgtatcgtcaaagtgatccaagcacactcatagttggagtcgtactccaaaggcggcaatgacgagtcagacagatactcgtcgacgtttaaaccatcatctaagggcctcaaaactacctcggaactgctgcgctgatctggacaccacagaggttccgagcactttaggttgcaccaaatgtcccaccaggtgcaggcagaaaacgctggaacagcgtgtacagtttgtcttaacaaaaagtgagggcgctgaggtcgagcagggtggtgtgacttgttatagcctttagagctgcgaaagcgcgtatggatttggctcatcaggccagattgagggtctgtggacacatgtcatgttagtgtacttcaatcgccccctggatatagccccgacaataggccgtggcctcatttttttgccttccgcacatttccattgctcggtacccacaccttgcttctcctgcacttgccaaccttaatactggtttacattgaccaacatcttacaagcggggggcttgtctagggtatatataaacagtggctctcccaatcggttgccagtctcttttttcctttctttccccacagattcgaaatctaaactacacatcacac

SEQ ID NO: 7 - DNA, 47 bp, synthetic construct
  misc_feature 1..47: note = AarI-removal 1
  source 1..47: mol_type = other DNA
agaagtatcctaccatctaccatctccgaaagaaactcgtcgattcc

SEQ ID NO: 8 - DNA, 47 bp, synthetic construct
  misc_feature 1..47: note = AarI-removal 2
  source 1..47: mol_type = other DNA
ggaatcgacgagtttctttcggagatggtagatggtaggatacttct

SEQ ID NO: 9 - DNA, 10706 bp, synthetic construct
  misc_feature 1..10706: note = pRF109
  source 1..10706: mol_type = other DNA
catggacaagaaatactccatcggcctggacattggaaccaactctgtcggctgggctgtcatcaccgacgagtacaaggtgccctccaagaaattcaaggtcctcggaaacaccgatcgacactccatcaagaaaaacctcattggtgccctgttgttcgattctggcgagactgccgaagctaccagactcaagcgaactgctcggcgacgttacacccgacggaagaaccgaatctgctacctgcaggagatcttttccaacgagatggccaaggtggacgattcgttctttcatcgactggaggaatccttcctcgtcgaggaagacaagaaacacgagcgtcatcccatctttggcaacattgtggacgaggttgcttaccacgagaagtatcctaccatctaccatctccgaaagaaactcgtcgattccaccgacaaggcggatctcagacttatctacctcgctctggcacacatgatcaagtttcgaggtcatttcctcatcgagggcgatctcaatcccgacaacagcgatgtggacaagctgttcattcagctcgttcagacctacaaccagctgttcgaggaaaaccccatcaatgcctccggagtcgatgcaaaggccatcttgtctgctcgactctcgaagagcagacgactggagaacctcattgcccaacttcctggcgagaaaaagaacggactgtttggcaacctcattgccctttctcttggtctcacacccaacttcaagtccaacttcgatctggcggaggacgccaagctccagctgtccaaggacacctacgacgatgacctcgacaacctgcttgcacagattggcgatcagtacgccgacctgtttctcgctgccaagaacctttcggatgctattctcttgtctgacattctgcgagtcaacaccgagatcacaaaggctcccctttctgcctccatgatcaagcgatacgacgagcaccatcaggatctcacactgctcaaggctcttgtccgacagcaactgcccgagaagtacaaggagatctttttcgatcagtcgaagaacggctacgctggatacatcgacggcggagcctctcaggaagagttctacaagttcatcaagccaattctcgagaagatggacggaaccgaggaactgcttgtcaagctcaatcgagaggatctgcttcggaagcaacgaaccttcgacaacggcagcattcctcatcagatccacctcggtgagctgcacgccattcttcgacgtcaggaagacttctacccctttctcaaggacaaccgagagaagatcgagaagattcttacctttcgaatcccctactatgttggtcctcttgccagaggaaactctcgatttgcttggatgactcgaaagtccgaggaaaccatcactccctggaacttcgaggaagtcgtggacaagggtgcctctgcacagtccttcatcgagcgaatgaccaacttcgacaagaatctgcccaacgagaaggttcttcccaagcattcgctgctctacgagtactttacagtctacaacgaactcaccaaagtcaagtacgttaccgagggaatgcgaaagcctgccttcttgtctggcgaacagaagaaagccattgtcgatctcctgttcaagaccaaccgaaaggtcactgttaagcagctcaaggaggactacttcaagaaaatcgagtgtttcgacagcgtcgagatttccggagttgaggaccgattcaacgcctctttgggcacctatcacgatctgctcaagattatcaaggacaaggattttctcgacaacgaggaaaacgaggacattctggaggacatcgtgctcactcttaccctgttcgaagatcgggagatgatcgaggaacgactcaagacatacgctcacctgttcgacgacaaggtcatgaaacaactcaagcgacgtagatacaccggctggggaagactttcgcgaaagctcatcaacggcatcagagacaagcagtccggaaagaccattctggactttctcaagtccgatggctttgccaaccgaaacttcatgcagctcattcacgacgattctcttaccttcaaggaggacatccagaaggcacaagtgtccggtcagggcgacagcttgcacgaacatattgccaacctggctggttcgccagccatcaagaaaggcattctccagactgtcaaggttgtcgacgagctggtgaaggtcatgggacgtcacaagcccgagaacattgtgatcgagatggccagagagaaccagacaactcaaaagggtcagaaaaactcgcgagagcggatgaagcgaatcgaggaaggcatcaaggagctgggatcccagattctcaaggagcatcccgtcgagaacactcaactgcagaacgagaagctgtatctctactatctgcagaatggtcgagacatgtacgtggatcaggaactggacatcaatcgtctcagcgactacgatgtggaccacattgtccctcaatcctttctcaaggacgattctatcgacaacaaggtccttacacgatccgacaagaacagaggcaagtcggacaacgttcccagcgaagaggtggtcaaaaagatgaagaactactggcgacagctgctcaacgccaagctcattacccagcgaaagttcgacaatcttaccaaggccgagcgaggcggtctgtccgagctcgacaaggctggcttcatcaagcgtcaactcgtcgagaccagacagatcacaaagcacgtcgcacagattctcgattctcggatgaacaccaagtacgacgagaacgacaagctcatccgagaggtcaaggtgattactctcaagtccaaactggtctccgatttccgaaaggactttcagttctacaaggtgcgagagatcaacaattaccaccatgcccacgatgcttacctcaacgccgtcgttggcactgcgctcatcaagaaataccccaagctcgaaagcgagttcgtttacggcgattacaaggtctacgacgttcgaaagatgattgccaagtccgaacaggagattggcaaggctactgccaagtacttcttttactccaacatcatgaactttttcaagaccgagatcaccttggccaacggagagattcgaaagagaccacttatcgagaccaacggcgaaactggagagatcgtgtgggacaagggtcgagactttgcaaccgtgcgaaaggttctgtcgatgcctcaggtcaacatcgtcaagaaaaccgaggttcagactggcggattctccaaggagtcgattctgcccaagcgaaactccgacaagctcatcgctcgaaagaaagactgggatcccaagaaatacggtggcttcgattctcctaccgtcgcctattccgtgcttgtcgttgcgaaggtcgagaagggcaagtccaaaaagctcaagtccgtcaaggagctgctcggaattaccatcatggagcgatcgagcttcgagaagaatcccatcgacttcttggaagccaagggttacaaggaggtcaagaaagacctcattatcaagctgcccaagtactctctgttcgaactggagaacggtcgaaagcgtatgctcgcctccgctggcgagctgcagaagggaaacgagcttgccttgccttcgaagtacgtcaactttctctatctggcttctcactacgagaagctcaagggttctcccgaggacaacgaacagaagcaactcttcgttgagcagcacaaacattacctcgacgagattatcgagcagatttccgagttttcgaagcgagtcatcctggctgatgccaacttggacaaggtgctctctgcctacaacaagcatcgggacaaacccattcgagaacaggcggagaacatcattcacctgtttactcttaccaacctgggtgctcctgcagctttcaagtacttcgataccactatcgaccgaaagcggtacacatccaccaaggaggttctcgatgccaccctgattcaccagtccatcactggcctgtacgagacccgaatcgacctgtctcagcttggtggcgactccagagccgatcccaagaaaaagcgaaaggtctaagcggccgcaagtgtggatggggaagtgagtgcccggttctgtgtgcacaattggcaatccaagatggatggattcaacacagggatatagcgagctacgtggtggtgcgaggatatagcaacggatatttatgtttgacacttgagaatgtacgatacaagcactgtccaagtacaatactaaacatactgtacatactcatactcgtacccgggcaacggtttcacttgagtgcagtggctagtgctcttactcgtacagtgtgcaatactgcgtatcatagtctttgatgtatatcgtattcattcatgttagttgcgtacgagccggaagcataaagtgtaaagcctggggtgcctaatgagtgagctaactcacattaattgcgttgcgctcactgcccgctttccagtcgggaaacctgtcgtgccagctgcattaatgaatcggccaacgcgcggggagaggcggtttgcgtattgggcgctcttccgcttcctcgctcactgactcgctgcgctcggtcgttcggctgcggcgagcggtatcagctcactcaaaggcggtaatacggttatccacagaatcaggggataacgcaggaaagaacatgtgagcaaaaggccagcaaaaggccaggaaccgtaaaaaggccgcgttgctggcgtttttccataggctccgcccccctgacgagcatcacaaaaatcgacgctcaagtcagaggtggcgaaacccgacaggactataaagataccaggcgtttccccctggaagctccctcgtgcgctctcctgttccgaccctgccgcttaccggatacctgtccgcctttctcccttcgggaagcgtggcgctttctcatagctcacgctgtaggtatctcagttcggtgtaggtcgttcgctccaagctgggctgtgtgcacgaaccccccgttcagcccgaccgctgcgccttatccggtaactatcgtcttgagtccaacccggtaagacacgacttatcgccactggcagcagccactggtaacaggattagcagagcgaggtatgtaggcggtgctacagagttcttgaagtggtggcctaactacggctacactagaaggacagtatttggtatctgcgctctgctgaagccagttaccttcggaaaaagagttggtagctcttgatccggcaaacaaaccaccgctggtagcggtggtttttttgtttgcaagcagcagattacgcgcagaaaaaaaggatctcaagaagatcctttgatcttttctacggggtctgacgctcagtggaacgaaaactcacgttaagggattttggtcatgagattatcaaaaaggatcttcacctagatccttttaaattaaaaatgaagttttaaatcaatctaaagtatatatgagtaaacttggtctgacagttaccaatgcttaatcagtgaggcacctatctcagcgatctgtctatttcgttcatccatagttgcctgactccccgtcgtgtagataactacgatacgggagggcttaccatctggccccagtgctgcaatgataccgcgagacccacgctcaccggctccagatttatcagcaataaaccagccagccggaagggccgagcgcagaagtggtcctgcaactttatccgcctccatccagtctattaattgttgccgggaagctagagtaagtagttcgccagttaatagtttgcgcaacgttgttgccattgctacaggcatcgtggtgtcacgctcgtcgtttggtatggcttcattcagctccggttcccaacgatcaaggcgagttacatgatcccccatgttgtgcaaaaaagcggttagctccttcggtcctccgatcgttgtcagaagtaagttggccgcagtgttatcactcatggttatggcagcactgcataattctcttactgtcatgccatccgtaagatgcttttctgtgactggtgagtactcaaccaagtcattctgagaatagtgtatgcggcgaccgagttgctcttgcccggcgtcaatacgggataataccgcgccacatagcagaactttaaaagtgctcatcattggaaaacgttcttcggggcgaaaactctcaaggatcttaccgctgttgagatccagttcgatgtaacccactcgtgcacccaactgatcttcagcatcttttactttcaccagcgtttctgggtgagcaaaaacaggaaggcaaaatgccgcaaaaaagggaataagggcgacacggaaatgttgaatactcatactcttcctttttcaatattattgaagcatttatcagggttattgtctcatgagcggatacatatttgaatgtatttagaaaaataaacaaataggggttccgcgcacatttccccgaaaagtgccacctgacgcgccctgtagcggcgcattaagcgcggcgggtgtggtggttacgcgcagcgtgaccgctacacttgccagcgccctagcgcccgctcctttcgctttcttcccttcctttctcgccacgttcgccggctttccccgtcaagctctaaatcgggggctccctttagggttccgatttagtgctttacggcacctcgaccccaaaaaacttgattagggtgatggttcacgtagtgggccatcgccctgatagacggtttttcgccctttgacgttggagtccacgttctttaatagtggactcttgttccaaactggaacaacactcaaccctatctcggtctattcttttgatttataagggattttgccgatttcggcctattggttaaaaaatgagctgatttaacaaaaatttaacgcgaattttaacaaaatattaacgcttacaatttccattcgccattcaggctgcgcaactgttgggaagggcgatcggtgcgggcctcttcgctattacgccagctggcgaaagggggatgtgctgcaaggcgattaagttgggtaacgccagggttttcccagtcacgacgttgtaaaacgacggccagtgaattgtaatacgactcactatagggcgaattgggtaccgggccccccctcgaggtcgatggtgtcgataagcttgatatcgaattcatgtcacacaaaccgatcttcgcctcaaggaaacctaattctacatccgagagactgccgagatccagtctacactgattaattttcgggccaataatttaaaaaaatcgtgttatataatattatatgtattatatatatacatcatgatgatactgacagtcatgtcccattgctaaatagacagactccatctgccgcctccaactgatgttctcaatatttaaggggtcatctcgcattgtttaataataaacagactccatctaccgcctccaaatgatgttctcaaaatatattgtatgaacttatttttattacttagtattattagacaacttacttgctttatgaaaaacacttcctatttaggaaacaatttataatggcagttcgttcatttaacaatttatgtagaataaatgttataaatgcgtatgggaaatcttaaatatggatagcataaatgatatctgcattgcctaattcgaaatcaacagcaacgaaaaaaatcccttgtacaacataaatagtcatcgagaaatatcaactatcaaagaacagctattcacacgttactattgagattattattggacgagaatcacacactcaactgtctttctctcttctagaaatacaggtacaagtatgtactattctcattgttcatacttctagtcatttcatcccacatattccttggatttctctccaatgaatgacattctatcttgcaaattcaacaattataataagatataccaaagtagcggtatagtggcaatcaaaaagcttctctggtgtgcttctcgtatttatttttattctaatgatccattaaaggtatatatttatttcttgttatataatccttttgtttattacatgggctggatacataaaggtattttgatttaattttttgcttaaattcaatcccccctcgttcagtgtcaactgtaatggtaggaaattaccatacttttgaagaagcaaaaaaaatgaaagaaaaaaaaaatcgtatttccaggttagacgttccgcagaatctagaatgcggtatgcggtacattgttcttcgaacgtaaaagttgcgctccctgagatattgtacatttttgcttttacaagtacaagtacatcgtacaactatgtactactgttgatgcatccacaacagtttgttttgtttttttttgttttttttttttctaatgattcattaccgctatgtatacctacttgtacttgtagtaagccgggttattggcgttcaattaatcatagacttatgaatctgcacggtgtgcgctgcgagttacttttagcttatgcatgctacttgggtgtaatattgggatctgttcggaaatcaacggatgctcaatcgatttcgacagtaattaattaagtcatacacaagtcagctttcttcgagcctcatataagtataagtagttcaacgtattagcactgtacccagcatctccgtatcgagaaacacaacaacatgccccattggacagatcatgcggatacacaggttgtgcagtatcatacatactcgatcagacaggtcgtctgaccatcatacaagctgaacaagcgctccatacttgcacgctctctatatacacagttaaattacatatccatagtctaacctctaacagttaatcttctggtaagcctcccagccagccttctggtatcgcttggcctcctcaataggatctcggttctggccgtacagacctcggccgacaattatgatatccgttccggtagacatgacatcctcaacagttcggtactgctgtccgagagcgtctcccttgtcgtcaagacccaccccgggggtcagaataagccagtcctcagagtcgcccttaggtcggttctgggcaatgaagccaaccacaaactcggggtcggatcgggcaagctcaatggtctgcttggagtactcgccagtggccagagagcccttgcaagacagctcggccagcatgagcagacctctggccagcttctcgttgggagaggggactaggaactccttgtactgggagttctcgtagtcagagacgtcctccttcttctgttcagagacagtttcctcggcaccagctcgcaggccagcaatgattccggttccgggtacaccgtgggcgttggtgatatcggaccactcggcgattcggtgacaccggtactggtgcttgacagtgttgccaatatctgcgaactttctgtcctcgaacaggaagaaaccgtgcttaagagcaagttccttgagggggagcacagtgccggcgtaggtgaagtcgtcaatgatgtcgatatgggttttgatcatgcacacataaggtccgaccttatcggcaagctcaatgagctccttggtggtggtaacatccagagaagcacacaggttggttttcttggctgccacgagcttgagcactcgagcggcaaaggcggacttgtggacgttagctcgagcttcgtaggagggcattttggtggtgaagaggagactgaaataaatttagtctgcagaactttttatcggaaccttatctggggcagtgaagtatatgttatggtaatagttacgagttagttgaacttatagatagactggactatacggctatcggtccaaattagaaagaacgtcaatggctctctgggcgtcgcctttgccgacaaaaatgtgatcatgatgaaagccagcaatgacgttgcagctgatattgttgtcggccaaccgcgccgaaaacgcagctgtcagacccacagcctccaacgaagaatgtatcgtcaaagtgatccaagcacactcatagttggagtcgtactccaaaggcggcaatgacgagtcagacagatactcgtcgacgtttaaaccatcatctaagggcctcaaaactacctcggaactgctgcgctgatctggacaccacagaggttccgagcactttaggttgcaccaaatgtcccaccaggtgcaggcagaaaacgctggaacagcgtgtacagtttgtcttaacaaaaagtgagggcgctgaggtcgagcagggtggtgtgacttgttatagcctttagagctgcgaaagcgcgtatggatttggctcatcaggccagattgagggtctgtggacacatgtcatgttagtgtacttcaatcgccccctggatatagccccgacaataggccgtggcctcatttttttgccttccgcacatttccattgctcggtacccacaccttgcttctcctgcacttgccaaccttaatactggtttacattgaccaacatcttacaagcggggggcttgtctagggtatatataaacagtggctctcccaatcggttgccagtctcttttttcctttctttccccacagattcgaaatctaaactacacatcacac

SEQ ID NO: 10 - DNA, 4140 bp, synthetic construct; identical to SEQ ID NO: 2
  misc_feature 1..4140: note = Aar1- Cas9 ORF
  source 1..4140: mol_type = other DNA

SEQ ID NO: 11 - DNA, 10706 bp, synthetic construct; identical to SEQ ID NO: 9
  misc_feature 1..10706: note = pRF141
  source 1..10706: mol_type = other DNA

SEQ ID NO: 12 - DNA, 1048 bp, synthetic construct
  misc_feature 1..1048: note = high-throughput cloning cassette
  source 1..1048: mol_type = other DNA
gcgcacgttaattaaattttttttgattttcttttttgaccccgtcttcaattacacttcccaactgggaacacccctctttatcgacccattttaggtaatttaccctagcccattgtctccataaggaatattaccctaacccacagtccagggtgcccaggtccttctttggccaaattttaacttcggtcctatggcacagcggtagcgcgtgagattgcaaatcttaaggtcccgagttcgaatctcggtgggacctagttatttttgatagataatttcgtgatgattagaaacttaacgcaaaataatggccggcatggtcccagcctcctcgctggcgccggctgggcaacatgcttcggcatggcgaatgggacgcaggtgatggcgggatcgttgtatatttcttgacaccttttcggcatcgccctaaattcggcgtcctcatattgtgtgaggacgttttattacgtgtttacgaagcaaaagctaaaaccaggagctatttaatggcaacagttaaccagctggtacgcaaaccacgtgctcgcaaagttgcgaaaagcaacgtgcctgcgctggaagcatgcccgcaaaaacgtggcgtatgtactcgtgtatatactaccactcctaaaaaaccgaactccgcgctgcgtaaagtatgccgtgttcgtctgactaacggtttcgaagtgacttcctacatcggtggtgaaggtcacaacctgcaggagcactccgtgatcctgatccgtggcggtcgtgttaaagacctcccgggtgttcgttaccacaccgtacgtggtgcgcttgactgctccggcgttaaagaccgtaagcaggctcgttccaagtatggcgtgaagcgtcctaaggcttaggttaataacaggcctgctggtaatcgcaggcctttttatttttacacctgcgttttagagctagaaatagcaagttaaaataaggctagtccgttatcaacttgaaaaagtggcaccgagtcggtgcttttttttttgttttttatcgatgcgcgcac

SEQ ID NO: 13 - DNA, 300 bp, Yarrowia lipolytica
  source 1..300: mol_type = genomic DNA
attttttttgattttcttttttgaccccgtcttcaattacacttcccaactgggaacacccctctttatcgacccattttaggtaatttaccctagcccattgtctccataaggaatattaccctaacccacagtccagggtgcccaggtccttctttggccaaattttaacttcggtcctatggcacagcggtagcgcgtgagattgcaaatcttaaggtcccgagttcgaatctcggtgggacctagttatttttgatagataatttcgtgatgattagaaacttaacgcaaaataat

SEQ ID NO: 14 - DNA, 68 bp, Herpes Delta virus
  source 1..68: mol_type = genomic DNA
ggccggcatggtcccagcctcctcgctggcgccggctgggcaacatgcttcggcatggcgaatgggac

SEQ ID NO: 15 - DNA, 544 bp, Escherischia coli
  source 1..544: mol_type = genomic DNA
atggcgggatcgttgtatatttcttgacaccttttcggcatcgccctaaattcggcgtcctcatattgtgtgaggacgttttattacgtgtttacgaagcaaaagctaaaaccaggagctatttaatggcaacagttaaccagctggtacgcaaaccacgtgctcgcaaagttgcgaaaagcaacgtgcctgcgctggaagcatgcccgcaaaaacgtggcgtatgtactcgtgtatatactaccactcctaaaaaaccgaactccgcgctgcgtaaagtatgccgtgttcgtctgactaacggtttcgaagtgacttcctacatcggtggtgaaggtcacaacctgcaggagcactccgtgatcctgatccgtggcggtcgtgttaaagacctcccgggtgttcgttaccacaccgtacgtggtgcgcttgactgctccggcgttaaagaccgtaagcaggctcgttccaagtatggcgtgaagcgtcctaaggcttaggttaataacaggcctgctggtaatcgcaggcctttttattttta

SEQ ID NO: 16 - DNA, 80 bp, synthetic construct
  misc_feature 1..80: note = DNA encoding Cas9 CER domain
  source 1..80: mol_type = other DNA
gttttagagctagaaatagcaagttaaaataaggctagtccgttatcaacttgaaaaagtggcaccgagtcggtgctttt

SEQ ID NO: 17 - DNA, 14 bp, Saccharomyces cerevisiae
  source 1..14: mol_type = genomic DNA
tttttttgtttttt

SEQ ID NO: 18 - DNA, 11714 bp, synthetic construct
  misc_feature 1..11714: note = pRF291
  source 1..11714: mol_type = other DNA
cgataaaaaacaaaaaaaaaagcaccgactcggtgccactttttcaagttgataacggactagccttattttaacttgctatttctagctctaaaacgcaggtgtaaaaataaaaaggcctgcgattaccagcaggcctgttattaacctaagccttaggacgcttcacgccatacttggaacgagcctgcttacggtctttaacgccggagcagtcaagcgcaccacgtacggtgtggtaacgaacacccgggaggtctttaacacgaccgccacggatcaggatcacggagtgctcctgcaggttgtgaccttcaccaccgatgtaggaagtcacttcgaaaccgttagtcagacgaacacggcatactttacgcagcgcggagttcggttttttaggagtggtagtatatacacgagtacatacgccacgtttttgcgggcatgcttccagcgcaggcacgttgcttttcgcaactttgcgagcacgtggtttgcgtaccagctggttaactgttgccattaaatagctcctggttttagcttttgcttcgtaaacacgtaataaaacgtcctcacacaatatgaggacgccgaatttagggcgatgccgaaaaggtgtcaagaaatatacaacgatcccgccatcacctgcgtcccattcgccatgccgaagcatgttgcccagccggcgccagcgaggaggctgggaccatgccggccattattttgcgttaagtttctaatcatcacgaaattatctatcaaaaataactaggtcccaccgagattcgaactcgggaccttaagatttgcaatctcacgcgctaccgctgtgccataggaccgaagttaaaatttggccaaagaaggacctgggcaccctggactgtgggttagggtaatattccttatggagacaatgggctagggtaaattacctaaaatgggtcgataaagaggggtgttcccagttgggaagtgtaattgaagacggggtcaaaaaagaaaatcaaaaaaaatttaattaagtcatacacaagtcagctttcttcgagcctcatataagtataagtagttcaacgtattagcactgtacccagcatctccgtatcgagaaacacaacaacatgccccattggacagatcatgcggatacacaggttgtgcagtatcatacatactcgatcagacaggtcgtctgaccatcatacaagctgaacaagcgctccatacttgcacgctctctatatacacagttaaattacatatccatagtctaacctctaacagttaatcttctggtaagcctcccagccagccttctggtatcgcttggcctcctcaataggatctcggttctggccgtacagacctcggccgacaattatgatatccgttccggtagacatgacatcctcaacagttcggtactgctgtccgagagcgtctcccttgtcgtcaagacccaccccgggggtcagaataagccagtcctcagagtcgcccttaggtcggttctgggcaatgaagccaaccacaaactcggggtcggatcgggcaagctcaatggtctgcttggagtactcgccagtggccagagagcccttgcaagacagctcggccagcatgagcagacctctggccagcttctcgttgggagaggggactaggaactccttgtactgggagttctcgtagtcagagacgtcctccttcttctgttcagagacagtttcctcggcaccagctcgcaggccagcaatgattccggttccgggtacaccgtgggcgttggtgatatcggaccactcggcgattcggtgacaccggtactggtgcttgacagtgttgccaatatctgcgaactttctgtcctcgaacaggaagaaaccgtgcttaagagcaagttccttgagggggagcacagtgccggcgtaggtgaagtcgtcaatgatgtcgatatgggttttgatcatgcacacataaggtccgaccttatcggcaagctcaatgagctccttggtggtggtaacatccagagaagcacacaggttggttttcttggctgccacgagcttgagcactcgagcggcaaaggcggacttgtggacgttagctcgagcttcgtaggagggcattttggtggtgaagaggagactgaaataaatttagtctgcagaactttttatcggaaccttatctggggcagtgaagtatatgttatggtaatagttacgagttagttgaacttatagatagactggactatacggctatcggtccaaattagaaagaacgtcaatggctctctgggcgtcgcctttgccgacaaaaatgtgatcatgatgaaagccagcaatgacgttgcagctgatattgttgtcggccaaccgcgccgaaaacgcagctgtcagacccacagcctccaacgaagaatgtatcgtcaaagtgatccaagcacactcatagttggagtcgtactccaaaggcggcaatgacgagtcagacagatactcgtcgacgtttaaaccatcatctaagggcctcaaaactacctcggaactgctgcgctgatctggacaccacagaggttccgagcactttaggttgcaccaaatgtcccaccaggtgcaggcagaaaacgctggaacagcgtgtacagtttgtcttaacaaaaagtgagggcgctgaggtcgagcagggtggtgtgacttgttatagcctttagagctgcgaaagcgcgtatggatttggctcatcaggccagattgagggtctgtggacacatgtcatgttagtgtacttcaatcgccccctggatatagccccgacaataggccgtggcctcatttttttgccttccgcacatttccattgctcggtacccacaccttgcttctcctgcacttgccaaccttaatactggtttacattgaccaacatcttacaagcggggggcttgtctagggtatatataaacagtggctctcccaatcggttgccagtctcttttttcctttctttccccacagattcgaaatctaaactacacatcacaccatggacaagaaatactccatcggcctggacattggaaccaactctgtcggctgggctgtcatcaccgacgagtacaaggtgccctccaagaaattcaaggtcctcggaaacaccgatcgacactccatcaagaaaaacctcattggtgccctgttgttcgattctggcgagactgccgaagctaccagactcaagcgaactgctcggcgacgttacacccgacggaagaaccgaatctgctacctgcaggagatcttttccaacgagatggccaaggtggacgattcgttctttcatcgactggaggaatccttcctcgtcgaggaagacaagaaacacgagcgtcatcccatctttggcaacattgtggacgaggttgcttaccacgagaagtatcctaccatctaccatctccgaaagaaactcgtcgattccaccgacaaggcggatctcagacttatctacctcgctctggcacacatgatcaagtttcgaggtcatttcctcatcgagggcgatctcaatcccgacaacagcgatgtggacaagctgttcattcagctcgttcagacctacaaccagctgttcgaggaaaaccccatcaatgcctccggagtcgatgcaaaggccatcttgtctgctcgactctcgaagagcagacgactggagaacctcattgcccaacttcctggcgagaaaaagaacggactgtttggcaacctcattgccctttctcttggtctcacacccaacttcaagtccaacttcgatctggcggaggacgccaagctccagctgtccaaggacacctacgacgatgacctcgacaacctgcttgcacagattggcgatcagtacgccgacctgtttctcgctgccaagaacctttcggatgctattctcttgtctgacattctgcgagtcaacaccgagatcacaaaggctcccctttctgcctccatgatcaagcgatacgacgagcaccatcaggatctcacactgctcaaggctcttgtccgacagcaactgcccgagaagtacaaggagatctttttcgatcagtcgaagaacggctacgctggatacatcgacggcggagcctctcaggaagagttctacaagttcatcaagccaattctcgagaagatggacggaaccgaggaactgcttgtcaagctcaatcgagaggatctgcttcggaagcaacgaaccttcgacaacggcagcattcctcatcagatccacctcggtgagctgcacgccattcttcgacgtcaggaagacttctacccctttctcaaggacaaccgagagaagatcgagaagattcttacctttcgaatcccctactatgttggtcctcttgccagaggaaactctcgatttgcttggatgactcgaaagtccgaggaaaccatcactccctggaacttcgaggaagtcgtggacaagggtgcctctgcacagtccttcatcgagcgaatgaccaacttcgacaagaatctgcccaacgagaaggttcttcccaagcattcgctgctctacgagtactttacagtctacaacgaactcaccaaagtcaagtacgttaccgagggaatgcgaaagcctgccttcttgtctggcgaacagaagaaagccattgtcgatctcctgttcaagaccaaccgaaaggtcactgttaagcagctcaaggaggactacttcaagaaaatcgagtgtttcgacagcgtcgagatttccggagttgaggaccgattcaacgcctctttgggcacctatcacgatctgctcaagattatcaaggacaaggattttctcgacaacgaggaaaacgaggacattctggaggacatcgtgctcactcttaccctgttcgaagatcgggagatgatcgaggaacgactcaagacatacgctcacctgttcgacgacaaggtcatgaaacaactcaagcgacgtagatacaccggctggggaagactttcgcgaaagctcatcaacggcatcagagacaagcagtccggaaagaccattctggactttctcaagtccgatggctttgccaaccgaaacttcatgcagctcattcacgacgattctcttaccttcaaggaggacatccagaaggcacaagtgtccggtcagggcgacagcttgcacgaacatattgccaacctggctggttcgccagccatcaagaaaggcattctccagactgtcaaggttgtcgacgagctggtgaaggtcatgggacgtcacaagcccgagaacattgtgatcgagatggccagagagaaccagacaactcaaaagggtcagaaaaactcgcgagagcggatgaagcgaatcgaggaaggcatcaaggagctgggatcccagattctcaaggagcatcccgtcgagaacactcaactgcagaacgagaagctgtatctctactatctgcagaatggtcgagacatgtacgtggatcaggaactggacatcaatcgtctcagcgactacgatgtggaccacattgtccctcaatcctttctcaaggacgattctatcgacaacaaggtccttacacgatccgacaagaacagaggcaagtcggacaacgttcccagcgaagaggtggtcaaaaagatgaagaactactggcgacagctgctcaacgccaagctcattacccagcgaaagttcgacaatcttaccaaggccgagcgaggcggtctgtccgagctcgacaaggctggcttcatcaagcgtcaactcgtcgagaccagacagatcacaaagcacgtcgcacagattctcgattctcggatgaacaccaagtacgacgagaacgacaagctcatccgagaggtcaaggtgattactctcaagtccaaactggtctccgatttccgaaaggactttcagttctacaaggtgcgagagatcaacaattaccaccatgcccacgatgcttacctcaacgccgtcgttggcactgcgctcatcaagaaataccccaagctcgaaagcgagttcgtttacggcgattacaaggtctacgacgttcgaaagatgattgccaagtccgaacaggagattggcaaggctactgccaagtacttcttttactccaacatcatgaactttttcaagaccgagatcaccttggccaacggagagattcgaaagagaccacttatcgagaccaacggcgaaactggagagatcgtgtgggacaagggtcgagactttgcaaccgtgcgaaaggttctgtcgatgcctcaggtcaacatcgtcaagaaaaccgaggttcagactggcggattctccaaggagtcgattctgcccaagcgaaactccgacaagctcatcgctcgaaagaaagactgggatcccaagaaatacggtggcttcgattctcctaccgtcgcctattccgtgcttgtcgttgcgaaggtcgagaagggcaagtccaaaaagctcaagtccgtcaaggagctgctcggaattaccatcatggagcgatcgagcttcgagaagaatcccatcgacttcttggaagccaagggttacaaggaggtcaagaaagacctcattatcaagctgcccaagtactctctgttcgaactggagaacggtcgaaagcgtatgctcgcctccgctggcgagctgcagaagggaaacgagcttgccttgccttcgaagtacgtcaactttctctatctggcttctcactacgagaagctcaagggttctcccgaggacaacgaacagaagcaactcttcgttgagcagcacaaacattacctcgacgagattatcgagcagatttccgagttttcgaagcgagtcatcctggctgatgccaacttggacaaggtgctctctgcctacaacaagcatcgggacaaacccattcgagaacaggcggagaacatcattcacctgtttactcttaccaacctgggtgctcctgcagctttcaagtacttcgataccactatcgaccgaaagcggtacacatccaccaaggaggttctcgatgccaccctgattcaccagtccatcactggcctgtacgagacccgaatcgacctgtctcagcttggtggcgactccagagccgatcccaagaaaaagcgaaaggtctaagcggccgcaagtgtggatggggaagtgagtgcccggttctgtgtgcacaattggcaatccaagatggatggattcaacacagggatatagcgagctacgtggtggtgcgaggatatagcaacggatatttatgtttgacacttgagaatgtacgatacaagcactgtccaagtacaatactaaacatactgtacatactcatactcgtacccgggcaacggtttcacttgagtgcagtggctagtgctcttactcgtacagtgtgcaatactgcgtatcatagtctttgatgtatatcgtattcattcatgttagttgcgtacgagccggaagcataaagtgtaaagcctggggtgcctaatgagtgagctaactcacattaattgcgttgcgctcactgcccgctttccagtcgggaaacctgtcgtgccagctgcattaatgaatcggccaacgcgcggggagaggcggtttgcgtattgggcgctcttccgcttcctcgctcactgactcgctgcgctcggtcgttcggctgcggcgagcggtatcagctcactcaaaggcggtaatacggttatccacagaatcaggggataacgcaggaaagaacatgtgagcaaaaggccagcaaaaggccaggaaccgtaaaaaggccgcgttgctggcgtttttccataggctccgcccccctgacgagcatcacaaaaatcgacgctcaagtcagaggtggcgaaacccgacaggactataaagataccaggcgtttccccctggaagctccctcgtgcgctctcctgttccgaccctgccgcttaccggatacctgtccgcctttctcccttcgggaagcgtggcgctttctcatagctcacgctgtaggtatctcagttcggtgtaggtcgttcgctccaagctgggctgtgtgcacgaaccccccgttcagcccgaccgctgcgccttatccggtaactatcgtcttgagtccaacccggtaagacacgacttatcgccactggcagcagccactggtaacaggattagcagagcgaggtatgtaggcggtgctacagagttcttgaagtggtggcctaactacggctacactagaaggacagtatttggtatctgcgctctgctgaagccagttaccttcggaaaaagagttggtagctcttgatccggcaaacaaaccaccgctggtagcggtggtttttttgtttgcaagcagcagattacgcgcagaaaaaaaggatctcaagaagatcctttgatcttttctacggggtctgacgctcagtggaacgaaaactcacgttaagggattttggtcatgagattatcaaaaaggatcttcacctagatccttttaaattaaaaatgaagttttaaatcaatctaaagtatatatgagtaaacttggtctgacagttaccaatgcttaatcagtgaggcacctatctcagcgatctgtctatttcgttcatccatagttgcctgactccccgtcgtgtagataactacgatacgggagggcttaccatctggccccagtgctgcaatgataccgcgagacccacgctcaccggctccagatttatcagcaataaaccagccagccggaagggccgagcgcagaagtggtcctgcaactttatccgcctccatccagtctattaattgttgccgggaagctagagtaagtagttcgccagttaatagtttgcgcaacgttgttgccattgctacaggcatcgtggtgtcacgctcgtcgtttggtatggcttcattcagctccggttcccaacgatcaaggcgagttacatgatcccccatgttgtgcaaaaaagcggttagctccttcggtcctccgatcgttgtcagaagtaagttggccgcagtgttatcactcatggttatggcagcactgcataattctcttactgtcatgccatccgtaagatgcttttctgtgactggtgagtactcaaccaagtcattctgagaatagtgtatgcggcgaccgagttgctcttgcccggcgtcaatacgggataataccgcgccacatagcagaactttaaaagtgctcatcattggaaaacgttcttcggggcgaaaactctcaaggatcttaccgctgttgagatccagttcgatgtaacccactcgtgcacccaactgatcttcagcatcttttactttcaccagcgtttctgggtgagcaaaaacaggaaggcaaaatgccgcaaaaaagggaataagggcgacacggaaatgttgaatactcatactcttcctttttcaatattattgaagcatttatcagggttattgtctcatgagcggatacatatttgaatgtatttagaaaaataaacaaataggggttccgcgcacatttccccgaaaagtgccacctgacgcgccctgtagcggcgcattaagcgcggcgggtgtggtggttacgcgcagcgtgaccgctacacttgccagcgccctagcgcccgctcctttcgctttcttcccttcctttctcgccacgttcgccggctttccccgtcaagctctaaatcgggggctccctttagggttccgatttagtgctttacggcacctcgaccccaaaaaacttgattagggtgatggttcacgtagtgggccatcgccctgatagacggtttttcgccctttgacgttggagtccacgttctttaatagtggactcttgttccaaactggaacaacactcaaccctatctcggtctattcttttgatttataagggattttgccgatttcggcctattggttaaaaaatgagctgatttaacaaaaatttaacgcgaattttaacaaaatattaacgcttacaatttccattcgccattcaggctgcgcaactgttgggaagggcgatcggtgcgggcctcttcgctattacgccagctggcgaaagggggatgtgctgcaaggcgattaagttgggtaacgccagggttttcccagtcacgacgttgtaaaacgacggccagtgaattgtaatacgactcactatagggcgaattgggtaccgggccccccctcgaggtcgatggtgtcgataagcttgatatcgaattcatgtcacacaaaccgatcttcgcctcaaggaaacctaattctacatccgagagactgccgagatccagtctacactgattaattttcgggccaataatttaaaaaaatcgtgttatataatattatatgtattatatatatacatcatgatgatactgacagtcatgtcccattgctaaatagacagactccatctgccgcctccaactgatgttctcaatatttaaggggtcatctcgcattgtttaataataaacagactccatctaccgcctccaaatgatgttctcaaaatatattgtatgaacttatttttattacttagtattattagacaacttacttgctttatgaaaaacacttcctatttaggaaacaatttataatggcagttcgttcatttaacaatttatgtagaataaatgttataaatgcgtatgggaaatcttaaatatggatagcataaatgatatctgcattgcctaattcgaaatcaacagcaacgaaaaaaatcccttgtacaacataaatagtcatcgagaaatatcaactatcaaagaacagctattcacacgttactattgagattattattggacgagaatcacacactcaactgtctttctctcttctagaaatacaggtacaagtatgtactattctcattgttcatacttctagtcatttcatcccacatattccttggatttctctccaatgaatgacattctatcttgcaaattcaacaattataataagatataccaaagtagcggtatagtggcaatcaaaaagcttctctggtgtgcttctcgtatttatttttattctaatgatccattaaaggtatatatttatttcttgttatataatccttttgtttattacatgggctggatacataaaggtattttgatttaattttttgcttaaattcaatcccccctcgttcagtgtcaactgtaatggtaggaaattaccatacttttgaagaagcaaaaaaaatgaaagaaaaaaaaaatcgtatttccaggttagacgttccgcagaatctagaatgcggtatgcggtacattgttcttcgaacgtaaaagttgcgctccctgagatattgtacatttttgcttttacaagtacaagtacatcgtacaactatgtactactgttgatgcatccacaacagtttgttttgtttttttttgttttttttttttctaatgattcattaccgctatgtatacctacttgtacttgtagtaagccgggttattggcgttcaattaatcatagacttatgaatctgcacggtgtgcgctgcgagttacttttagcttatgcatgctacttgggtgtaatattgggatctgttcggaaatcaacggatgctcaat

SEQ ID NO: 19 - DNA, 32 bp, synthetic construct
  misc_feature 1..32: note = Can1-1F
  source 1..32: mol_type = other DNA
aatgggactcaaacgattacccaccctcgttt

SEQ ID NO: 20 - DNA, 32 bp, synthetic construct
  misc_feature 1..32: note = Can1-1R
  source 1..32: mol_type = other DNA
tctaaaacgagggtgggtaatcgtttgagtcc

SEQ ID NO: 21 - DNA, 20 bp, synthetic construct
  misc_feature 1..20: note = DNA encoding Can1-1 VT domain
  source 1..20: mol_type = other DNA
tcaaacgattacccaccctc

SEQ ID NO: 22 - DNA, 23 bp, Yarrowia lipolytica
  source 1..23: mol_type = genomic DNA
tcaaacgattacccaccctccgg

SEQ ID NO: 23 - DNA, 1719 bp, Yarrowia lipolytica
  source 1..1719: mol_type = genomic DNA
atggaaaagacattttcaaacgattacccaccctccgggactgaggcccacatccacatcaaccacacggcccactcggatgactcagaggaggtgccctcgcacaaggaaaattacaacaccagtggccacgacctggaggagtccgacccggataaccatgtcggtgagaccctcgaggtcaagcgaggtctcaagatgcgacacatctccatgatctcgcttggaggaaccattggtaccggtctcttcattggtaccggaggagctctccagcaggccggtccctgtggcgccctcgtcgcctacgtgttcatggccaccattgtctactctgttgccgagtctcttggagaactggctacgtacattcccatcaccggctcctttgccgtctttactacccgatatctgtcacagtcgtttggtgcctccatgggctggctatactggttctcgtgggcgatcaccttcgccatcgagctcaacaccattggtcccgtgattgagtactggactgacgccgttcctactgctgcctggattgccatcttcttcgtcatcctcactaccatcaacttcttccccgtgggcttctatggcgaagtcgagttctgggtggcctccgtgaaggtcattgccatcattggatggctcatctacgcgctctgcatgacgtgtggagcaggtgtaacaggtcctgtgggattcagatactggaaccaccccggacccatgggagacggaatctggaccgacggcgtgcccattgtgcgaaacgcgcccggtcgacgattcatgggatggctcaattcgctcgttaacgccgccttcacctaccagggctgtgagctggtcggagtcactgccggtgaggcccagaaccccagaaagtccgtccctcgagccatcaaccgagtctttgctcgaatttgcatcttctacattggctctatcttcttcatgggcatgctcgtgccctttaacgaccccaagctgaccgatgactcctccgtcatcgcctcctctccttttgttattgccattatcaactctggcaccaaggtgctccctcacattttcaacgccgtcattctcatcaccctgatttcggcaggaaactccaacgtctacattggctcgcgagtggtctacgccctggctgactccggaaccgcaccaaagttcttcaagcgaaccaccaagaagggagtgccgtacgtggcagtctgcttcacctcggcgtttggtctgctggccttcatgtctgtgtccgagtcgtcgtccactgtcttcgactggttcatcaacatctccgctgtggccggcctcatctgttgggccttcatctctgcctcccacatccgattcatgcaagtgcttaagcacagagggatctccagagatacgctgcccttcaaggcacgatggcagccattctactcatggtacgcgctcgtctccatcatcttcatcactctcatccagggcttcacgtccttctggcactttaccgccgccaagttcatgactgcatacatctccgtcattgtctgggtcggtttgtacattatcttccagtgtctgttccgatgcaagttccttatccctattgaggatgtggacattgacaccggccgacgagagattgacgacgatgtgtgggaggagaagatccccacaaagtggtacgagaagttttggaatattattgcataa

SEQ ID NO: 24 - DNA, 11176 bp, synthetic construct
  misc_feature 1..11176: note = pRF303
  source 1..11176: mol_type = other DNA
tctaaaacgagggtgggtaatcgtttgagtcccattcgccatgccgaagcatgttgcccagccggcgccagcgaggaggctgggaccatgccggccattattttgcgttaagtttctaatcatcacgaaattatctatcaaaaataactaggtcccaccgagattcgaactcgggaccttaagatttgcaatctcacgcgctaccgctgtgccataggaccgaagttaaaatttggccaaagaaggacctgggcaccctggactgtgggttagggtaatattccttatggagacaatgggctagggtaaattacctaaaatgggtcgataaagaggggtgttcccagttgggaagtgtaattgaagacggggtcaaaaaagaaaatcaaaaaaaatttaattaagtcatacacaagtcagctttcttcgagcctcatataagtataagtagttcaacgtattagcactgtacccagcatctccgtatcgagaaacacaacaacatgccccattggacagatcatgcggatacacaggttgtgcagtatcatacatactcgatcagacaggtcgtctgaccatcatacaagctgaacaagcgctccatacttgcacgctctctatatacacagttaaattacatatccatagtctaacctctaacagttaatcttctggtaagcctcccagccagccttctggtatcgcttggcctcctcaataggatctcggttctggccgtacagacctcggccgacaattatgatatccgttccggtagacatgacatcctcaacagttcggtactgctgtccgagagcgtctcccttgtcgtcaagacccaccccgggggtcagaataagccagtcctcagagtcgcccttaggtcggttctgggcaatgaagccaaccacaaactcggggtcggatcgggcaagctcaatggtctgcttggagtactcgccagtggccagagagcccttgcaagacagctcggccagcatgagcagacctctggccagcttctcgttgggagaggggactaggaactccttgtactgggagttctcgtagtcagagacgtcctccttcttctgttcagagacagtttcctcggcaccagctcgcaggccagcaatgattccggttccgggtacaccgtgggcgttggtgatatcggaccactcggcgattcggtgacaccggtactggtgcttgacagtgttgccaatatctgcgaactttctgtcctcgaacaggaagaaaccgtgcttaagagcaagttccttgagggggagcacagtgccggcgtaggtgaagtcgtcaatgatgtcgatatgggttttgatcatgcacacataaggtccgaccttatcggcaagctcaatgagctccttggtggtggtaacatccagagaagcacacaggttggttttcttggctgccacgagcttgagcactcgagcggcaaaggcggacttgtggacgttagctcgagcttcgtaggagggcattttggtggtgaagaggagactgaaataaatttagtctgcagaactttttatcggaaccttatctggggcagtgaagtatatgttatggtaatagttacgagttagttgaacttatagatagactggactatacggctatcggtccaaattagaaagaacgtcaatggctctctgggcgtcgcctttgccgacaaaaatgtgatcatgatgaaagccagcaatgacgttgcagctgatattgttgtcggccaaccgcgccgaaaacgcagctgtcagacccacagcctccaacgaagaatgtatcgtcaaagtgatccaagcacactcatagttggagtcgtactccaaaggcggcaatgacgagtcagacagatactcgtcgacgtttaaaccatcatctaagggcctcaaaactacctcggaactgctgcgctgatctggacaccacagaggttccgagcactttaggttgcaccaaatgtcccaccaggtgcaggcagaaaacgctggaacagcgtgtacagtttgtcttaacaaaaagtgagggcgctgaggtcgagcagggtggtgtgacttgttatagcctttagagctgcgaaagcgcgtatggatttggctcatcaggccagattgagggtctgtggacacatgtcatgttagtgtacttcaatcgccccctggatatagccccgacaataggccgtggcctcatttttttgccttccgcacatttccattgctcggtacccacaccttgcttctcctgcacttgccaaccttaatactggtttacattgaccaacatcttacaagcggggggcttgtctagggtatatataaacagtggctctcccaatcggttgccagtctcttttttcctttctttccccacagattcgaaatctaaactacacatcacaccatggacaagaaatactccatcggcctggacattggaaccaactctgtcggctgggctgtcatcaccgacgagtacaaggtgccctccaagaaattcaaggtcctcggaaacaccgatcgacactccatcaagaaaaacctcattggtgccctgttgttcgattctggcgagactgccgaagctaccagactcaagcgaactgctcggcgacgttacacccgacggaagaaccgaatctgctacctgcaggagatcttttccaacgagatggccaaggtggacgattcgttctttcatcgactggaggaatccttcctcgtcgaggaagacaagaaacacgagcgtcatcccatctttggcaacattgtggacgaggttgcttaccacgagaagtatcctaccatctaccatctccgaaagaaactcgtcgattccaccgacaaggcggatctcagacttatctacctcgctctggcacacatgatcaagtttcgaggtcatttcctcatcgagggcgatctcaatcccgacaacagcgatgtggacaagctgttcattcagctcgttcagacctacaaccagctgttcgaggaaaaccccatcaatgcctccggagtcgatgcaaaggccatcttgtctgctcgactctcgaagagcagacgactggagaacctcattgcccaacttcctggcgagaaaaagaacggactgtttggcaacctcattgccctttctcttggtctcacacccaacttcaagtccaacttcgatctggcggaggacgccaagctccagctgtccaaggacacctacgacgatgacctcgacaacctgcttgcacagattggcgatcagtacgccgacctgtttctcgctgccaagaacctttcggatgctattctcttgtctgacattctgcgagtcaacaccgagatcacaaaggctcccctttctgcctccatgatcaagcgatacgacgagcaccatcaggatctcacactgctcaaggctcttgtccgacagcaactgcccgagaagtacaaggagatctttttcgatcagtcgaagaacggctacgctggatacatcgacggcggagcctctcaggaagagttctacaagttcatcaagccaattctcgagaagatggacggaaccgaggaactgcttgtcaagctcaatcgagaggatctgcttcggaagcaacgaaccttcgacaacggcagcattcctcatcagatccacctcggtgagctgcacgccattcttcgacgtcaggaagacttctacccctttctcaaggacaaccgagagaagatcgagaagattcttacctttcgaatcccctactatgttggtcctcttgccagaggaaactctcgatttgcttggatgactcgaaagtccgaggaaaccatcactccctggaacttcgaggaagtcgtggacaagggtgcctctgcacagtccttcatcgagcgaatgaccaacttcgacaagaatctgcccaacgagaaggttcttcccaagcattcgctgctctacgagtactttacagtctacaacgaactcaccaaagtcaagtacgttaccgagggaatgcgaaagcctgccttcttgtctggcgaacagaagaaagccattgtcgatctcctgttcaagaccaaccgaaaggtcactgttaagcagctcaaggaggactacttcaagaaaatcgagtgtttcgacagcgtcgagatttccggagttgaggaccgattcaacgcctctttgggcacctatcacgatctgctcaagattatcaaggacaaggattttctcgacaacgaggaaaacgaggacattctggaggacatcgtgctcactcttaccctgttcgaagatcgggagatgatcgaggaacgactcaagacatacgctcacctgttcgacgacaaggtcatgaaacaactcaagcgacgtagatacaccggctggggaagactttcgcgaaagctcatcaacggcatcagagacaagcagtccggaaagaccattctggactttctcaagtccgatggctttgccaaccgaaacttcatgcagctcattcacgacgattctcttaccttcaaggaggacatccagaaggcacaagtgtccggtcagggcgacagcttgcacgaacatattgccaacctggctggttcgccagccatcaagaaaggcattctccagactgtcaaggttgtcgacgagctggtgaaggtcatgggacgtcacaagcccgagaacattgtgatcgagatggccagagagaaccagacaactcaaaagggtcagaaaaactcgcgagagcggatgaagcgaatcgaggaaggcatcaaggagctgggatcccagattctcaaggagcatcccgtcgagaacactcaactgcagaacgagaagctgtatctctactatctgcagaatggtcgagacatgtacgtggatcaggaactggacatcaatcgtctcagcgactacgatgtggaccacattgtccctcaatcctttctcaaggacgattctatcgacaacaaggtccttacacgatccgacaagaacagaggcaagtcggacaacgttcccagcgaagaggtggtcaaaaagatgaagaactactggcgacagctgctcaacgccaagctcattacccagcgaaagttcgacaatcttaccaaggccgagcgaggcggtctgtccgagctcgacaaggctggcttcatcaagcgtcaactcgtcgagaccagacagatcacaaagcacgtcgcacagattctcgattctcggatgaacaccaagtacgacgagaacgacaagctcatccgagaggtcaaggtgattactctcaagtccaaactggtctccgatttccgaaaggactttcagttctacaaggtgcgagagatcaacaattaccaccatgcccacgatgcttacctcaacgccgtcgttggcactgcgctcatcaagaaataccccaagctcgaaagcgagttcgtttacggcgattacaaggtctacgacgttcgaaagatgattgccaagtccgaacaggagattggcaaggctactgccaagtacttcttttactccaacatcatgaactttttcaagaccgagatcaccttggccaacggagagattcgaaagagaccacttatcgagaccaacggcgaaactggagagatcgtgtgggacaagggtcgagactttgcaaccgtgcgaaaggttctgtcgatgcctcaggtcaacatcgtcaagaaaaccgaggttcagactggcggattctccaaggagtcgattctgcccaagcgaaactccgacaagctcatcgctcgaaagaaagactgggatcccaagaaatacggtggcttcgattctcctaccgtcgcctattccgtgcttgtcgttgcgaaggtcgagaagggcaagtccaaaaagctcaagtccgtcaaggagctgctcggaattaccatcatggagcgatcgagcttcgagaagaatcccatcgacttcttggaagccaagggttacaaggaggtcaagaaagacctcattatcaagctgcccaagtactctctgttcgaactggagaacggtcgaaagcgtatgctcgcctccgctggcgagctgcagaagggaaacgagcttgccttgccttcgaagtacgtcaactttctctatctggcttctcactacgagaagctcaagggttctcccgaggacaacgaacagaagcaactcttcgttgagcagcacaaacattacctcgacgagattatcgagcagatttccgagttttcgaagcgagtcatcctggctgatgccaacttggacaaggtgctctctgcctacaacaagcatcgggacaaacccattcgagaacaggcggagaacatcattcacctgtttactcttaccaacctgggtgctcctgcagctttcaagtacttcgataccactatcgaccgaaagcggtacacatccaccaaggaggttctcgatgccaccctgattcaccagtccatcactggcctgtacgagacccgaatcgacctgtctcagcttggtggcgactccagagccgatcccaagaaaaagcgaaaggtctaagcggccgcaagtgtggatggggaagtgagtgcccggttctgtgtgcacaattggcaatccaagatggatggattcaacacagggatatagcgagctacgtggtggtgcgaggatatagcaacggatatttatgtttgacacttgagaatgtacgatacaagcactgtccaagtacaatactaaacatactgtacatactcatactcgtacccgggcaacggtttcacttgagtgcagtggctagtgctcttactcgtacagtgtgcaatactgcgtatcatagtctttgatgtatatcgtattcattcatgttagttgcgtacgagccggaagcataaagtgtaaagcctggggtgcctaatgagtgagctaactcacattaattgcgttgcgctcactgcccgctttccagtcgggaaacctgtcgtgccagctgcattaatgaatcggccaacgcgcggggagaggcggtttgcgtattgggcgctcttccgcttcctcgctcactgactcgctgcgctcggtcgttcggctgcggcgagcggtatcagctcactcaaaggcggtaatacggttatccacagaatcaggggataacgcaggaaagaacatgtgagcaaaaggccagcaaaaggccaggaaccgtaaaaaggccgcgttgctggcgtttttccataggctccgcccccctgacgagcatcacaaaaatcgacgctcaagtcagaggtggcgaaacccgacaggactataaagataccaggcgtttccccctggaagctccctcgtgcgctctcctgttccgaccctgccgcttaccggatacctgtccgcctttctcccttcgggaagcgtggcgctttctcatagctcacgctgtaggtatctcagttcggtgtaggtcgttcgctccaagctgggctgtgtgcacgaaccccccgttcagcccgaccgctgcgccttatccggtaactatcgtcttgagtccaacccggtaagacacgacttatcgccactggcagcagccactggtaacaggattagcagagcgaggtatgtaggcggtgctacagagttcttgaagtggtggcctaactacggctacactagaaggacagtatttggtatctgcgctctgctgaagccagttaccttcggaaaaagagttggtagctcttgatccggcaaacaaaccaccgctggtagcggtggtttttttgtttgcaagcagcagattacgcgcagaaaaaaaggatctcaagaagatcctttgatcttttctacggggtctgacgctcagtggaacgaaaactcacgttaagggattttggtcatgagattatcaaaaaggatcttcacctagatccttttaaattaaaaatgaagttttaaatcaatctaaagtatatatgagtaaacttggtctgacagttaccaatgcttaatcagtgaggcacctatctcagcgatctgtctatttcgttcatccatagttgcctgactccccgtcgtgtagataactacgatacgggagggcttaccatctggccccagtgctgcaatgataccgcgagacccacgctcaccggctccagatttatcagcaataaaccagccagccggaagggccgagcgcagaagtggtcctgcaactttatccgcctccatccagtctattaattgttgccgggaagctagagtaagtagttcgccagttaatagtttgcgcaacgttgttgccattgctacaggcatcgtggtgtcacgctcgtcgtttggtatggcttcattcagctccggttcccaacgatcaaggcgagttacatgatcccccatgttgtgcaaaaaagcggttagctccttcggtcctccgatcgttgtcagaagtaagttggccgcagtgttatcactcatggttatggcagcactgcataattctcttactgtcatgccatccgtaagatgcttttctgtgactggtgagtactcaaccaagtcattctgagaatagtgtatgcggcgaccgagttgctcttgcccggcgtcaatacgggataataccgcgccacatagcagaactttaaaagtgctcatcattggaaaacgttcttcggggcgaaaactctcaaggatcttaccgctgttgagatccagttcgatgtaacccactcgtgcacccaactgatcttcagcatcttttactttcaccagcgtttctgggtgagcaaaaacaggaaggcaaaatgccgcaaaaaagggaataagggcgacacggaaatgttgaatactcatactcttcctttttcaatattattgaagcatttatcagggttattgtctcatgagcggatacatatttgaatgtatttagaaaaataaacaaataggggttccgcgcacatttccccgaaaagtgccacctgacgcgccctgtagcggcgcattaagcgcggcgggtgtggtggttacgcgcagcgtgaccgctacacttgccagcgccctagcgcccgctcctttcgctttcttcccttcctttctcgccacgttcgccggctttccccgtcaagctctaaatcgggggctccctttagggttccgatttagtgctttacggcacctcgaccccaaaaaacttgattagggtgatggttcacgtagtgggccatcgccctgatagacggtttttcgccctttgacgttggagtccacgttctttaatagtggactcttgttccaaactggaacaacactcaaccctatctcggtctattcttttgatttataagggattttgccgatttcggcctattggttaaaaaatgagctgatttaacaaaaatttaacgcgaattttaacaaaatattaacgcttacaatttccattcgccattcaggctgcgcaactgttgggaagggcgatcggtgcgggcctcttcgctattacgccagctggcgaaagggggatgtgctgcaaggcgattaagttgggtaacgccagggttttcccagtcacgacgttgtaaaacgacggccagtgaattgtaatacgactcactatagggcgaattgggtaccgggccccccctcgaggtcgatggtgtcgataagcttgatatcgaattcatgtcacacaaaccgatcttcgcctcaaggaaacctaattctacatccgagagactgccgagatccagtctacactgattaattttcgggccaataatttaaaaaaatcgtgttatataatattatatgtattatatatatacatcatgatgatactgacagtcatgtcccattgctaaatagacagactccatctgccgcctccaactgatgttctcaatatttaaggggtcatctcgcattgtttaataataaacagactccatctaccgcctccaaatgatgttctcaaaatatattgtatgaacttatttttattacttagtattattagacaacttacttgctttatgaaaaacacttcctatttaggaaacaatttataatggcagttcgttcatttaacaatttatgtagaataaatgttataaatgcgtatgggaaatcttaaatatggatagcataaatgatatctgcattgcctaattcgaaatcaacagcaacgaaaaaaatcccttgtacaacataaatagtcatcgagaaatatcaactatcaaagaacagctattcacacgttactattgagattattattggacgagaatcacacactcaactgtctttctctcttctagaaatacaggtacaagtatgtactattctcattgttcatacttctagtcatttcatcccacatattccttggatttctctccaatgaatgacattctatcttgcaaattcaacaattataataagatataccaaagtagcggtatagtggcaatcaaaaagcttctctggtgtgcttctcgtatttatttttattctaatgatccattaaaggtatatatttatttcttgttatataatccttttgtttattacatgggctggatacataaaggtattttgatttaattttttgcttaaattcaatcccccctcgttcagtgtcaactgtaatggtaggaaattaccatacttttgaagaagcaaaaaaaatgaaagaaaaaaaaaatcgtatttccaggttagacgttccgcagaatctagaatgcggtatgcggtacattgttcttcgaacgtaaaagttgcgctccctgagatattgtacatttttgcttttacaagtacaagtacatcgtacaactatgtactactgttgatgcatccacaacagtttgttttgtttttttttgttttttttttttctaatgattcattaccgctatgtatacctacttgtacttgtagtaagccgggttattggcgttcaattaatcatagacttatgaatctgcacggtgtgcgctgcgagttacttttagcttatgcatgctacttgggtgtaatattgggatctgttcggaaatcaacggatgctcaatcgataaaaaacaaaaaaaaaagcaccgactcggtgccactttttcaagttgataacggactagccttattttaacttgctatttctagc

SEQ ID NO: 25 - DNA, 655 bp, synthetic construct
  misc_feature 1..655: note = can1 upstream homology arm
  source 1..655: mol_type = other DNA
gggaagccttgctacgttaggagaagacgcacggcgatgatacgggtacccctcatgacatcaatatccgctgcccctcttgccagcaaggcgtcagcaggtgcttttttcgctattttcaccagaccacagcctttttccttgtgtctcatcttggattccttcaaaggcaactcaccgcacctccgagtcgtgtgaacaatgtaataataggctattgacttttttcccacctgtttagcgccaaacccaaagcgcttttcgcccccactgcagcccgatggaaggcacatatggcaagggaaaagtcttcaggtaatacatgcctgctgcaactatatgtactctgactcattccctcagacgtgggtcatagacagctgttttaaaccgggcaaatcaatctctgtcgcacaggtatttctgcccttcaaaaccaggttgccacatcagattccatcaaagtttttcagactaacttcaatcttaaacggcatctcacaacaagcgaattggacggaaaaaaagcgtctatcattaccggcacctatccacactaagacagtactaaaggacgacgctccccacgaaacgacgtttcgaccttaacgaccctgccgtctccatccatccgaccactcccgacgctctctcc

SEQ ID NO: 26 - DNA, 29 bp, synthetic construct
  misc_feature 1..29: note = Can1 upstream forward
  source 1..29: mol_type = other DNA
gggaagcttgctacgttaggagaagacgc

SEQ ID NO: 27 - DNA, 37 bp, synthetic construct
  misc_feature 1..37: note = Can1 upstream reverse
  source 1..37: mol_type = other DNA
ggagagagcgtcgggagtggtcggatggatggagacg

SEQ ID NO: 28 - DNA, 658 bp, synthetic construct
  misc_feature 1..658: note = Can1 downstream homology arm
  source 1..658: mol_type = other DNA
cgtctccatccatccgaccactcccgacgctctctcctggagcaaaccactcttaccaagcatatagcatatataataacgtattgaatttattaactgattgaattgagagtaaagccagtagcgttgtacggctgtagctttttagaaaagtggcagatgagcgatggtggatatgaaagtacctttacggcatgtagcgacacaagatcgcttccaagaactcgacattcaagcccagctcgtacaagaaaatgaactagccaatcatatgaactagcacattgaagtcaccgcatcatctctgttggaaacgacgcgcatgtactcgtgcgtagtaaatccgtatctgtacactcgaaagattacagtatgtagtagtagcatgactaacgatgtaacgtccaaataacgctctgtgcctactcctgtagatgcattagaccacctgctaacgtctacacgttatgtccgttagctccaagattgcacttttccctcaaagactctgctgggttacgtcatggtctctttcgggtctctggtccgttctctgcccgcccatatccgcccaggctgctacgatacaggataagctcataagcttagattatttttccggaatgacatcacgatgcagtggtggaaggatgtatgg

SEQ ID NO: 29 - DNA, 37 bp, synthetic construct
  misc_feature 1..37: note = Can1 downstream homology arm forward primer
  source 1..37: mol_type = other DNA
cgtctccatccatccgaccactcccgacgctctctcc

SEQ ID NO: 30 - DNA, 22 bp, Yarrowia lipolytica
  source 1..22: mol_type = genomic DNA
ccatacatccttccaccactgc

SEQ ID NO: 31 - DNA, 1276 bp, synthetic construct
  misc_feature 1..1276: note = Can1 editing template clonign fragment
  source 1..1276: mol_type = other DNA
gggaagccttgctacgttaggagaagacgcacggcgatgatacgggtacccctcatgacatcaatatccgctgcccctcttgccagcaaggcgtcagcaggtgcttttttcgctattttcaccagaccacagcctttttccttgtgtctcatcttggattccttcaaaggcaactcaccgcacctccgagtcgtgtgaacaatgtaataataggctattgacttttttcccacctgtttagcgccaaacccaaagcgcttttcgcccccactgcagcccgatggaaggcacatatggcaagggaaaagtcttcaggtaatacatgcctgctgcaactatatgtactctgactcattccctcagacgtgggtcatagacagctgttttaaaccgggcaaatcaatctctgtcgcacaggtatttctgcccttcaaaaccaggttgccacatcagattccatcaaagtttttcagactaacttcaatcttaaacggcatctcacaacaagcgaattggacggaaaaaaagcgtctatcattaccggcacctatccacactaagacagtactaaaggacgacgctccccacgaaacgacgtttcgaccttaacgaccctgccgtctccatccatccgaccactcccgacgctctctcctggagcaaaccactcttaccaagcatatagcatatataataacgtattgaatttattaactgattgaattgagagtaaagccagtagcgttgtacggctgtagctttttagaaaagtggcagatgagcgatggtggatatgaaagtacctttacggcatgtagcgacacaagatcgcttccaagaactcgacattcaagcccagctcgtacaagaaaatgaactagccaatcatatgaactagcacattgaagtcaccgcatcatctctgttggaaacgacgcgcatgtactcgtgcgtagtaaatccgtatctgtacactcgaaagattacagtatgtagtagtagcatgactaacgatgtaacgtccaaataacgctctgtgcctactcctgtagatgcattagaccacctgctaacgtctacacgttatgtccgttagctccaagattgcacttttccctcaaagactctgctgggttacgtcatggtctctttcgggtctctggtccgttctctgcccgcccatatccgcccaggctgctacgatacaggataagctcataagcttagattatttttccggaatgacatcacgatgcagtggtggaaggatgtatgg

SEQ ID NO: 32 - DNA, 2686 bp, synthetic construct
  misc_feature 1..2686: note = pUC18
  source 1..2686: mol_type = other DNA
tcgcgcgtttcggtgatgacggtgaaaacctctgacacatgcagctcccggagacggtcacagcttgtctgtaagcggatgccgggagcagacaagcccgtcagggcgcgtcagcgggtgttggcgggtgtcggggctggcttaactatgcggcatcagagcagattgtactgagagtgcaccatatgcggtgtgaaataccgcacagatgcgtaaggagaaaataccgcatcaggcgccattcgccattcaggctgcgcaactgttgggaagggcgatcggtgcgggcctcttcgctattacgccagctggcgaaagggggatgtgctgcaaggcgattaagttgggtaacgccagggttttcccagtcacgacgttgtaaaacgacggccagtgccaagcttgcatgcctgcaggtcgactctagaggatccccgggtaccgagctcgaattcgtaatcatggtcatagctgtttcctgtgtgaaattgttatccgctcacaattccacacaacatacgagccggaagcataaagtgtaaagcctggggtgcctaatgagtgagctaactcacattaattgcgttgcgctcactgcccgctttccagtcgggaaacctgtcgtgccagctgcattaatgaatcggccaacgcgcggggagaggcggtttgcgtattgggcgctcttccgcttcctcgctcactgactcgctgcgctcggtcgttcggctgcggcgagcggtatcagctcactcaaaggcggtaatacggttatccacagaatcaggggataacgcaggaaagaacatgtgagcaaaaggccagcaaaaggccaggaaccgtaaaaaggccgcgttgctggcgtttttccataggctccgcccccctgacgagcatcacaaaaatcgacgctcaagtcagaggtggcgaaacccgacaggactataaagataccaggcgtttccccctggaagctccctcgtgcgctctcctgttccgaccctgccgcttaccggatacctgtccgcctttctcccttcgggaagcgtggcgctttctcatagctcacgctgtaggtatctcagttcggtgtaggtcgttcgctccaagctgggctgtgtgcacgaaccccccgttcagcccgaccgctgcgccttatccggtaactatcgtcttgagtccaacccggtaagacacgacttatcgccactggcagcagccactggtaacaggattagcagagcgaggtatgtaggcggtgctacagagttcttgaagtggtggcctaactacggctacactagaaggacagtatttggtatctgcgctctgctgaagccagttaccttcggaaaaagagttggtagctcttgatccggcaaacaaaccaccgctggtagcggtggtttttttgtttgcaagcagcagattacgcgcagaaaaaaaggatctcaagaagatcctttgatcttttctacggggtctgacgctcagtggaacgaaaactcacgttaagggattttggtcatgagattatcaaaaaggatcttcacctagatccttttaaattaaaaatgaagttttaaatcaatctaaagtatatatgagtaaacttggtctgacagttaccaatgcttaatcagtgaggcacctatctcagcgatctgtctatttcgttcatccatagttgcctgactccccgtcgtgtagataactacgatacgggagggcttaccatctggccccagtgctgcaatgataccgcgagacccacgctcaccggctccagatttatcagcaataaaccagccagccggaagggccgagcgcagaagtggtcctgcaactttatccgcctccatccagtctattaattgttgccgggaagctagagtaagtagttcgccagttaatagtttgcgcaacgttgttgccattgctacaggcatcgtggtgtcacgctcgtcgtttggtatggcttcattcagctccggttcccaacgatcaaggcgagttacatgatcccccatgttgtgcaaaaaagcggttagctccttcggtcctccgatcgttgtcagaagtaagttggccgcagtgttatcactcatggttatggcagcactgcataattctcttactgtcatgccatccgtaagatgcttttctgtgactggtgagtactcaaccaagtcattctgagaatagtgtatgcggcgaccgagttgctcttgcccggcgtcaatacgggataataccgcgccacatagcagaactttaaaagtgctcatcattggaaaacgttcttcggggcgaaaactctcaaggatcttaccgctgttgagatccagttcgatgtaacccactcgtgcacccaactgatcttcagcatcttttactttcaccagcgtttctgggtgagcaaaaacaggaaggcaaaatgccgcaaaaaagggaataagggcgacacggaaatgttgaatactcatactcttcctttttcaatattattgaagcatttatcagggttattgtctcatgagcggatacatatttgaatgtatttagaaaaataaacaaataggggttccgcgcacatttccccgaaaagtgccacctgacgtctaagaaaccattattatcatgacattaacctataaaaataggcgtatcacgaggccctttcgtc

SEQ ID NO: 33 - DNA, 3901 bp, synthetic construct
  misc_feature 1..3901: note = pRF80
  source 1..3901: mol_type = other DNA
agcttgctacgttaggagaagacgcacggcgatgatacgggtacccctcatgacatcaatatccgctgcccctcttgccagcaaggcgtcagcaggtgcttttttcgctattttcaccagaccacagcctttttccttgtgtctcatcttggattccttcaaaggcaactcaccgcacctccgagtcgtgtgaacaatgtaataataggctattgacttttttcccacctgtttagcgccaaacccaaagcgcttttcgcccccactgcagcccgatggaaggcacatatggcaagggaaaagtcttcaggtaatacatgcctgctgcaactatatgtactctgactcattccctcagacgtgggtcatagacagctgttttaaaccgggcaaatcaatctctgtcgcacaggtatttctgcccttcaaaaccaggttgccacatcagattccatcaaagtttttcagactaacttcaatcttaaacggcatctcacaacaagcgaattggacggaaaaaaagcgtctatcattaccggcacctatccacactaagacagtactaaaggacgacgctccccacgaaacgacgtttcgaccttaacgaccctgccgtctccatccatccgaccactcccgacgctctctcctggagcaaaccactcttaccaagcatatagcatatataataacgtattgaatttattaactgattgaattgagagtaaagccagtagcgttgtacggctgtagctttttagaaaagtggcagatgagcgatggtggatatgaaagtacctttacggcatgtagcgacacaagatcgcttccaagaactcgacattcaagcccagctcgtacaagaaaatgaactagccaatcatatgaactagcacattgaagtcaccgcatcatctctgttggaaacgacgcgcatgtactcgtgcgtagtaaatccgtatctgtacactcgaaagattacagtatgtagtagtagcatgactaacgatgtaacgtccaaataacgctctgtgcctactcctgtagatgcattagaccacctgctaacgtctacacgttatgtccgttagctccaagattgcacttttccctcaaagactctgctgggttacgtcatggtctctttcgggtctctggtccgttctctgcccgcccatatccgcccaggctgctacgatacaggataagctcataagcttgcatgcctgcaggtcgactctagaggatccccgggtaccgagctcgaattcgtaatcatggtcatagctgtttcctgtgtgaaattgttatccgctcacaattccacacaacatacgagccggaagcataaagtgtaaagcctggggtgcctaatgagtgagctaactcacattaattgcgttgcgctcactgcccgctttccagtcgggaaacctgtcgtgccagctgcattaatgaatcggccaacgcgcggggagaggcggtttgcgtattgggcgctcttccgcttcctcgctcactgactcgctgcgctcggtcgttcggctgcggcgagcggtatcagctcactcaaaggcggtaatacggttatccacagaatcaggggataacgcaggaaagaacatgtgagcaaaaggccagcaaaaggccaggaaccgtaaaaaggccgcgttgctggcgtttttccataggctccgcccccctgacgagcatcacaaaaatcgacgctcaagtcagaggtggcgaaacccgacaggactataaagataccaggcgtttccccctggaagctccctcgtgcgctctcctgttccgaccctgccgcttaccggatacctgtccgcctttctcccttcgggaagcgtggcgctttctcatagctcacgctgtaggtatctcagttcggtgtaggtcgttcgctccaagctgggctgtgtgcacgaaccccccgttcagcccgaccgctgcgccttatccggtaactatcgtcttgagtccaacccggtaagacacgacttatcgccactggcagcagccactggtaacaggattagcagagcgaggtatgtaggcggtgctacagagttcttgaagtggtggcctaactacggctacactagaaggacagtatttggtatctgcgctctgctgaagccagttaccttcggaaaaagagttggtagctcttgatccggcaaacaaaccaccgctggtagcggtggtttttttgtttgcaagcagcagattacgcgcagaaaaaaaggatctcaagaagatcctttgatcttttctacggggtctgacgctcagtggaacgaaaactcacgttaagggattttggtcatgagattatcaaaaaggatcttcacctagatccttttaaattaaaaatgaagttttaaatcaatctaaagtatatatgagtaaacttggtctgacagttaccaatgcttaatcagtgaggcacctatctcagcgatctgtctatttcgttcatccatagttgcctgactccccgtcgtgtagataactacgatacgggagggcttaccatctggccccagtgctgcaatgataccgcgagacccacgctcaccggctccagatttatcagcaataaaccagccagccggaagggccgagcgcagaagtggtcctgcaactttatccgcctccatccagtctattaattgttgccgggaagctagagtaagtagttcgccagttaatagtttgcgcaacgttgttgccattgctacaggcatcgtggtgtcacgctcgtcgtttggtatggcttcattcagctccggttcccaacgatcaaggcgagttacatgatcccccatgttgtgcaaaaaagcggttagctccttcggtcctccgatcgttgtcagaagtaagttggccgcagtgttatcactcatggttatggcagcactgcataattctcttactgtcatgccatccgtaagatgcttttctgtgactggtgagtactcaaccaagtcattctgagaatagtgtatgcggcgaccgagttgctcttgcccggcgtcaatacgggataataccgcgccacatagcagaactttaaaagtgctcatcattggaaaacgttcttcggggcgaaaactctcaaggatcttaccgctgttgagatccagttcgatgtaacccactcgtgcacccaactgatcttcagcatcttttactttcaccagcgtttctgggtgagcaaaaacaggaaggcaaaatgccgcaaaaaagggaataagggcgacacggaaatgttgaatactcatactcttcctttttcaatattattgaagcatttatcagggttattgtctcatgagcggatacatatttgaatgtatttagaaaaataaacaaataggggttccgcgcacatttccccgaaaagtgccacctgacgtctaagaaaccattattatcatgacattaacctataaaaataggcgtatcacgaggccctttcgtctcgcgcgtttcggtgatgacggtgaaaacctctgacacatgcagctcccggagacggtcacagcttgtctgtaagcggatgccgggagcagacaagcccgtcagggcgcgtcagcgggtgttggcgggtgtcggggctggcttaactatgcggcatcagagcagattgtactgagagtgcaccatatgcggtgtgaaataccgcacagatgcgtaaggagaaaataccgcatcaggcgccattcgccattcaggctgcgcaactgttgggaagggcgatcggtgcgggcctcttcgctattacgccagctggcgaaagggggatgtgctgcaaggcgattaagttgggtaacgccagggttttcccagtcacgacgttgtaaaacgacggccagtgcca

SEQ ID NO: 34 - DNA, 1210 bp, synthetic construct
  misc_feature 1..1210: note = Can1 polynucleotide modification (editing) template
  source 1..1210: mol_type = other DNA
gctacgttaggagaagacgcacggcgatgatacgggtacccctcatgacatcaatatccgctgcccctcttgccagcaaggcgtcagcaggtgcttttttcgctattttcaccagaccacagcctttttccttgtgtctcatcttggattccttcaaaggcaactcaccgcacctccgagtcgtgtgaacaatgtaataataggctattgacttttttcccacctgtttagcgccaaacccaaagcgcttttcgcccccactgcagcccgatggaaggcacatatggcaagggaaaagtcttcaggtaatacatgcctgctgcaactatatgtactctgactcattccctcagacgtgggtcatagacagctgttttaaaccgggcaaatcaatctctgtcgcacaggtatttctgcccttcaaaaccaggttgccacatcagattccatcaaagtttttcagactaacttcaatcttaaacggcatctcacaacaagcgaattggacggaaaaaaagcgtctatcattaccggcacctatccacactaagacagtactaaaggacgacgctccccacgaaacgacgtttcgaccttaacgaccctgccgtctccatccatccgaccactcccgacgctctctcctggagcaaaccactcttaccaagcatatagcatatataataacgtattgaatttattaactgattgaattgagagtaaagccagtagcgttgtacggctgtagctttttagaaaagtggcagatgagcgatggtggatatgaaagtacctttacggcatgtagcgacacaagatcgcttccaagaactcgacattcaagcccagctcgtacaagaaaatgaactagccaatcatatgaactagcacattgaagtcaccgcatcatctctgttggaaacgacgcgcatgtactcgtgcgtagtaaatccgtatctgtacactcgaaagattacagtatgtagtagtagcatgactaacgatgtaacgtccaaataacgctctgtgcctactcctgtagatgcattagaccacctgctaacgtctacacgttatgtccgttagctccaagattgcacttttccctcaaagactctgctgggttacgtcatggtctctttcgggtctctggtccgttctctgcccgcccatatccgcccaggctgctacgatacaggataagctcata

SEQ ID NO: 35 - DNA, 20 bp, synthetic construct
  misc_feature 1..20: note = C3S forward
  source 1..20: mol_type = other DNA
agcttgctacgttaggagaa

SEQ ID NO: 36 - DNA, 20 bp, synthetic construct
  misc_feature 1..20: note = C3S reverse
  source 1..20: mol_type = other DNA
tatgagcttatcctgtatcg

SEQ ID NO: 37 - DNA, 20 bp, synthetic construct
  misc_feature 1..20: note = PT forward
  source 1..20: mol_type = other DNA
agcttgctacgttaggagaa

SEQ ID NO: 38 - DNA, 20 bp, synthetic construct
  misc_feature 1..20: note = PT reverse
  source 1..20: mol_type = other DNA
tatgagcttatcctgtatcg

SEQ ID NO: 39 - DNA, 2125 bp, synthetic construct
  misc_feature 1..2125: note = CAN1 locus
  source 1..2125: mol_type = other DNA
ggaaggcacatatggcaagggaaaagtcttcaggtaatacatgcctgctgcaactatatgtactctgactcattccctcagacgtgggtcatagacagctgttttaaaccgggcaaatcaatctctgtcgcacaggtatttctgcccttcaaaaccaggttgccacatcagattccatcaaagtttttcagactaacttcaatcttaaacggcatctcacaacaagcgaattggacggaaaaaaagcgtctatcattaccggcacctatccacactaagacagtactaaaggacgacgctccccacgaaacgacgtttcgaccttaacgaccctgccgtctccatccatccgaccacaatggaaaagacattttcaaacgattacccaccctccgggactgaggcccacatccacatcaaccacacggcccactcggatgactcagaggaggtgccctcgcacaaggaaaattacaacaccagtggccacgacctggaggagtccgacccggataaccatgtcggtgagaccctcgaggtcaagcgaggtctcaagatgcgacacatctccatgatctcgcttggaggaaccattggtaccggtctcttcattggtaccggaggagctctccagcaggccggtccctgtggcgccctcgtcgcctacgtgttcatggccaccattgtctactctgttgccgagtctcttggagaactggctacgtacattcccatcaccggctcctttgccgtctttactacccgatatctgtcacagtcgtttggtgcctccatgggctggctatactggttctcgtgggcgatcaccttcgccatcgagctcaacaccattggtcccgtgattgagtactggactgacgccgttcctactgctgcctggattgccatcttcttcgtcatcctcactaccatcaacttcttccccgtgggcttctatggcgaagtcgagttctgggtggcctccgtgaaggtcattgccatcattggatggctcatctacgcgctctgcatgacgtgtggagcaggtgtaacaggtcctgtgggattcagatactggaaccaccccggacccatgggagacggaatctggaccgacggcgtgcccattgtgcgaaacgcgcccggtcgacgattcatgggatggctcaattcgctcgttaacgccgccttcacctaccagggctgtgagctggtcggagtcactgccggtgaggcccagaaccccagaaagtccgtccctcgagccatcaaccgagtctttgctcgaatttgcatcttctacattggctctatcttcttcatgggcatgctcgtgccctttaacgaccccaagctgaccgatgactcctccgtcatcgcctcctctccttttgttattgccattatcaactctggcaccaaggtgctccctcacattttcaacgccgtcattctcatcaccctgatttcggcaggaaactccaacgtctacattggctcgcgagtggtctacgccctggctgactccggaaccgcaccaaagttcttcaagcgaaccaccaagaagggagtgccgtacgtggcagtctgcttcacctcggcgtttggtctgctggccttcatgtctgtgtccgagtcgtcgtccactgtcttcgactggttcatcaacatctccgctgtggccggcctcatctgttgggccttcatctctgcctcccacatccgattcatgcaagtgcttaagcacagagggatctccagagatacgctgcccttcaaggcacgatggcagccattctactcatggtacgcgctcgtctccatcatcttcatcactctcatccagggcttcacgtccttctggcactttaccgccgccaagttcatgactgcatacatctccgtcattgtctgggtcggtttgtacattatcttccagtgtctgttccgatgcaagttccttatccctattgaggatgtggacattgacaccggccgacgagagattgacgacgatgtgtgggaggagaagatccccacaaagtggtacgagaagttttggaatattattgcataagaagatcggggattcccgacgctctctcctggagcaaaccactcttac

SEQ ID NO: 40 - DNA, 20 bp, synthetic construct
  misc_feature 1..20: note = unmodified forward
  source 1..20: mol_type = other DNA
agcttgctacgttaggagaa

SEQ ID NO: 41 - DNA, 20 bp, synthetic construct
  misc_feature 1..20: note = unmodified reverse
  source 1..20: mol_type = other DNA
tatgagcttatcctgtatcg

SEQ ID NO: 42 - DNA, 20 bp, Yarrowia lipolytica
  source 1..20: mol_type = genomic DNA
ggaaggcacatatggcaagg

SEQ ID NO: 43 - DNA, 21 bp, Yarrowia lipolytica
  source 1..21: mol_type = genomic DNA
gtaagagtggtttgctccagg

SEQ ID NO: 44 - DNA, 2125 bp, Yarrowia lipolytica; identical to SEQ ID NO: 39
  source 1..2125: mol_type = genomic DNA

SEQ ID NO: 45 - DNA, 392 bp, synthetic construct
  misc_feature 1..392: note = Can1 locus deletion
  source 1..392: mol_type = other DNA
ggaaggcacatatggcaagggaaaagtcttcaggtaatacatgcctgctgcaactatatgtactctgactcattccctcagacgtgggtcatagacagctgttttaaaccgggcaaatcaatctctgtcgcacaggtatttctgcccttcaaaaccaggttgccacatcagattccatcaaagtttttcagactaacttcaatcttaaacggcatctcacaacaagcgaattggacggaaaaaaagcgtctatcattaccggcacctatccacactaagacagtactaaaggacgacgctccccacgaaacgacgtttcgaccttaacgaccctgccgtctccatccatccgaccactcccgacgctctctcctggagcaaaccactcttac

SEQ ID NO: 46 - DNA, 62 bp, Yarrowia lipolytica
  misc_feature 1..62: note = Copy number analysis fragment
  source 1..62: mol_type = genomic DNA
agcgccaaacccaaagcgcttttcgcccccactgcagcccgatggaaggcacatatggcaag

SEQ ID NO: 47 - DNA, 17 bp, synthetic construct
  misc_feature 1..17: note = Can1 copy number F
  source 1..17: mol_type = other DNA
agcgccaaacccaaagc

SEQ ID NO: 48 - DNA, 20 bp, synthetic construct
  misc_feature 1..20: note = Can1 copy number R
  source 1..20: mol_type = other DNA
cttgccatatgtgccttcca

SEQ ID NO: 49 - DNA, 21 bp, synthetic construct
  misc_feature 1..21: note = Can1 copy number probe
  source 1..21: mol_type = other DNA
cttttcgcccccactgcagcc

SEQ ID NO: 50 - DNA, 69 bp, Yarrowia lipolytica
  source 1..69: mol_type = genomic DNA
tgaccgtccttggagataccagcctcgaactcaccaacaccaccagcaatgatgaggatggcacagtcg

SEQ ID NO: 51 - DNA, 20 bp, synthetic construct
  misc_feature 1..20: note = TEF1 forward
  source 1..20: mol_type = other DNA
cgactgtgccatcctcatca

SEQ ID NO: 52 - DNA, 21 bp, synthetic construct
  misc_feature 1..21: note = TEF1 reverse
  source 1..21: mol_type = other DNA
tgaccgtccttggagatacca

SEQ ID NO: 53 - DNA, 21 bp, Yarrowia lipolytica
  source 1..21: mol_type = genomic DNA
tgctggtggtgttggtgagtt

SEQ ID NO: 54 - DNA, 12167 bp, synthetic construct
  misc_feature 1..12167: note = pRF434
  source 1..12167: mol_type = other DNA
cgataaaaaacaaaaaaaaaagcaccgactcggtgccactttttcaagttgataacggactagccttattttaacttgctatttctagctctaaaacgcaggtgtaaaaataaaaaggcctgcgattaccagcaggcctgttattaacctaagccttaggacgcttcacgccatacttggaacgagcctgcttacggtctttaacgccggagcagtcaagcgcaccacgtacggtgtggtaacgaacacccgggaggtctttaacacgaccgccacggatcaggatcacggagtgctcctgcaggttgtgaccttcaccaccgatgtaggaagtcacttcgaaaccgttagtcagacgaacacggcatactttacgcagcgcggagttcggttttttaggagtggtagtatatacacgagtacatacgccacgtttttgcgggcatgcttccagcgcaggcacgttgcttttcgcaactttgcgagcacgtggtttgcgtaccagctggttaactgttgccattaaatagctcctggttttagcttttgcttcgtaaacacgtaataaaacgtcctcacacaatatgaggacgccgaatttagggcgatgccgaaaaggtgtcaagaaatatacaacgatcccgccatcacctgcgtcccattcgccatgccgaagcatgttgcccagccggcgccagcgaggaggctgggaccatgccggccattattttgcgttaagtttctaatcatcacgaaattatctatcaaaaataactaggtcccaccgagattcgaactcgggaccttaagatttgcaatctcacgcgctaccgctgtgccataggaccgaagttaaaatttggccaaagaaggacctgggcaccctggactgtgggttagggtaatattccttatggagacaatgggctagggtaaattacctaaaatgggtcgataaagaggggtgttcccagttgggaagtgtaattgaagacggggtcaaaaaagaaaatcaaaaaaaatttaattaagactatgataacttcgtataatgtatgctatacgaacggtagcacactgtacgagtaagagcactagccactgcactcaagtgaaaccgttgcccgggtacgagtatgagtatgtacagtatgtttagtattgtacttggacagtgcttgtatcgtacattctcaagtgtcaaacataaatatccgttgctatatcctcgcaccaccacgtagctcgctatatccctgtgttgaatccatccatcttggattgccaattgtgcacacagaaccgggcactcacttccccatccacacttgcggccgctattcctttgccctcggacgagtgctggggcgtcggtttccactatcggcgagtacttctacacagccatcggtccagacggccgcgcttctgcgggcgatttgtgtacgcccgacagtcccggctccggatcggacgattgcgtcgcatcgaccctgcgcccaagctgcatcatcgaaattgccgtcaaccaagctctgatagagttggtcaagaccaatgcggagcatatacgcccggagccgcggcgatcctgcaagctccggatgcctccgctcgaagtagcgcgtctgctgctccatacaagccaaccacggcctccagaagaagatgttggcgacctcgtattgggaatccccgaacatcgcctcgctccagtcaatgaccgctgttatgcggccattgtccgtcaggacattgttggagccgaaatccgcgtgcacgaggtgccggacttcggggcagtcctcggcccaaagcatcagctcatcgagagcctgcgcgacggacgcactgacggtgtcgtccatcacagtttgccagtgatacacatggggatcagcaatcgcgcatatgaaatcacgccatgtagtgtattgaccgattccttgcggtccgaatgggccgaacccgctcgtctggctaagatcggccgcagcgatcgcatccatagcctccgcgaccggctgcagaacagcgggcagttcggtttcaggcaggtcttgcaacgtgacaccctgtgcacggcgggagatgcaataggtcaggctctcgctgaactccccaatgtcaagcacttccggaatcgggagcgcggccgatgcaaagtgccgataaacataacgatctttgtagaaaccatcggcgcagctatttacccgcaggacatatccacgccctcctacatcgaagctgaaagcacgagattcttcgccctccgagagctgcatcaggtcggagacgctgtcgaacttttcgatcagaaacttctcgacagacgtcgcggtgagttcaggctttttggccatggttgatgtgtgtttaattcaagaatgaatatagagaagagaagaagaaaaaagattcaattgagccggcgatgcagacccttatataaatgttgccttggacagacggagcaagcccgcccaaacctacgttcggtataatatgttaagctttttaacacaaaggtttggcttggggtaacctgatgtggtgcaaaagaccgggcgttggcgagccattgcgcgggcgaatggggccgtgactcgtctcaaattcgagggcgtgcctcaattcgtgcccccgtggctttttcccgccgtttccgccccgtttgcaccactgcagccgcttctttggttcggacaccttgctgcgagctaggtgccttgtgctacttaaaaagtggcctcccaacaccaacatgacatgagtgcgtgggccaagacacgttggcggggtcgcagtcggctcaatggcccggaaaaaacgctgctggagctggttcggacgcagtccgccgcggcgtatggatatccgcaaggttccatagcgccattgccctccgtcggcgtctatcccgcaacctaccgttcgtataatgtatgctatacgaagttatgagcgggcttaaggtttaaaccatcatctaagggcctcaaaactacctcggaactgctgcgctgatctggacaccacagaggttccgagcactttaggttgcaccaaatgtcccaccaggtgcaggcagaaaacgctggaacagcgtgtacagtttgtcttaacaaaaagtgagggcgctgaggtcgagcagggtggtgtgacttgttatagcctttagagctgcgaaagcgcgtatggatttggctcatcaggccagattgagggtctgtggacacatgtcatgttagtgtacttcaatcgccccctggatatagccccgacaataggccgtggcctcatttttttgccttccgcacatttccattgctcggtacccacaccttgcttctcctgcacttgccaaccttaatactggtttacattgaccaacatcttacaagcggggggcttgtctagggtatatataaacagtggctctcccaatcggttgccagtctcttttttcctttctttccccacagattcgaaatctaaactacacatcacaccatggacaagaaatactccatcggcctggacattggaaccaactctgtcggctgggctgtcatcaccgacgagtacaaggtgccctccaagaaattcaaggtcctcggaaacaccgatcgacactccatcaagaaaaacctcattggtgccctgttgttcgattctggcgagactgccgaagctaccagactcaagcgaactgctcggcgacgttacacccgacggaagaaccgaatctgctacctgcaggagatcttttccaacgagatggccaaggtggacgattcgttctttcatcgactggaggaatccttcctcgtcgaggaagacaagaaacacgagcgtcatcccatctttggcaacattgtggacgaggttgcttaccacgagaagtatcctaccatctaccatctccgaaagaaactcgtcgattccaccgacaaggcggatctcagacttatctacctcgctctggcacacatgatcaagtttcgaggtcatttcctcatcgagggcgatctcaatcccgacaacagcgatgtggacaagctgttcattcagctcgttcagacctacaaccagctgttcgaggaaaaccccatcaatgcctccggagtcgatgcaaaggccatcttgtctgctcgactctcgaagagcagacgactggagaacctcattgcccaacttcctggcgagaaaaagaacggactgtttggcaacctcattgccctttctcttggtctcacacccaacttcaagtccaacttcgatctggcggaggacgccaagctccagctgtccaaggacacctacgacgatgacctcgacaacctgcttgcacagattggcgatcagtacgccgacctgtttctcgctgccaagaacctttcggatgctattctcttgtctgacattctgcgagtcaacaccgagatcacaaaggctcccctttctgcctccatgatcaagcgatacgacgagcaccatcaggatctcacactgctcaaggctcttgtccgacagcaactgcccgagaagtacaaggagatctttttcgatcagtcgaagaacggctacgctggatacatcgacggcggagcctctcaggaagagttctacaagttcatcaagccaattctcgagaagatggacggaaccgaggaactgcttgtcaagctcaatcgagaggatctgcttcggaagcaacgaaccttcgacaacggcagcattcctcatcagatccacctcggtgagctgcacgccattcttcgacgtcaggaagacttctacccctttctcaaggacaaccgagagaagatcgagaagattcttacctttcgaatcccctactatgttggtcctcttgccagaggaaactctcgatttgcttggatgactcgaaagtccgaggaaaccatcactccctggaacttcgaggaagtcgtggacaagggtgcctctgcacagtccttcatcgagcgaatgaccaacttcgacaagaatctgcccaacgagaaggttcttcccaagcattcgctgctctacgagtactttacagtctacaacgaactcaccaaagtcaagtacgttaccgagggaatgcgaaagcctgccttcttgtctggcgaacagaagaaagccattgtcgatctcctgttcaagaccaaccgaaaggtcactgttaagcagctcaaggaggactacttcaagaaaatcgagtgtttcgacagcgtcgagatttccggagttgaggaccgattcaacgcctctttgggcacctatcacgatctgctcaagattatcaaggacaaggattttctcgacaacgaggaaaacgaggacattctggaggacatcgtgctcactcttaccctgttcgaagatcgggagatgatcgaggaacgactcaagacatacgctcacctgttcgacgacaaggtcatgaaacaactcaagcgacgtagatacaccggctggggaagactttcgcgaaagctcatcaacggcatcagagacaagcagtccggaaagaccattctggactttctcaagtccgatggctttgccaaccgaaacttcatgcagctcattcacgacgattctcttaccttcaaggaggacatccagaaggcacaagtgtccggtcagggcgacagcttgcacgaacatattgccaacctggctggttcgccagccatcaagaaaggcattctccagactgtcaaggttgtcgacgagctggtgaaggtcatgggacgtcacaagcccgagaacattgtgatcgagatggccagagagaaccagacaactcaaaagggtcagaaaaactcgcgagagcggatgaagcgaatcgaggaaggcatcaaggagctgggatcccagattctcaaggagcatcccgtcgagaacactcaactgcagaacgagaagctgtatctctactatctgcagaatggtcgagacatgtacgtggatcaggaactggacatcaatcgtctcagcgactacgatgtggaccacattgtccctcaatcctttctcaaggacgattctatcgacaacaaggtccttacacgatccgacaagaacagaggcaagtcggacaacgttcccagcgaagaggtggtcaaaaagatgaagaactactggcgacagctgctcaacgccaagctcattacccagcgaaagttcgacaatcttaccaaggccgagcgaggcggtctgtccgagctcgacaaggctggcttcatcaagcgtcaactcgtcgagaccagacagatcacaaagcacgtcgcacagattctcgattctcggatgaacaccaagtacgacgagaacgacaagctcatccgagaggtcaaggtgattactctcaagtccaaactggtctccgatttccgaaaggactttcagttctacaaggtgcgagagatcaacaattaccaccatgcccacgatgcttacctcaacgccgtcgttggcactgcgctcatcaagaaataccccaagctcgaaagcgagttcgtttacggcgattacaaggtctacgacgttcgaaagatgattgccaagtccgaacaggagattggcaaggctactgccaagtacttcttttactccaacatcatgaactttttcaagaccgagatcaccttggccaacggagagattcgaaagagaccacttatcgagaccaacggcgaaactggagagatcgtgtgggacaagggtcgagactttgcaaccgtgcgaaaggttctgtcgatgcctcaggtcaacatcgtcaagaaaaccgaggttcagactggcggattctccaaggagtcgattctgcccaagcgaaactccgacaagctcatcgctcgaaagaaagactgggatcccaagaaatacggtggcttcgattctcctaccgtcgcctattccgtgcttgtcgttgcgaaggtcgagaagggcaagtccaaaaagctcaagtccgtcaaggagctgctcggaattaccatcatggagcgatcgagcttcgagaagaatcccatcgacttcttggaagccaagggttacaaggaggtcaagaaagacctcattatcaagctgcccaagtactctctgttcgaactggagaacggtcgaaagcgtatgctcgcctccgctggcgagctgcagaagggaaacgagcttgccttgccttcgaagtacgtcaactttctctatctggcttctcactacgagaagctcaagggttctcccgaggacaacgaacagaagcaactcttcgttgagcagcacaaacattacctcgacgagattatcgagcagatttccgagttttcgaagcgagtcatcctggctgatgccaacttggacaaggtgctctctgcctacaacaagcatcgggacaaacccattcgagaacaggcggagaacatcattcacctgtttactcttaccaacctgggtgctcctgcagctttcaagtacttcgataccactatcgaccgaaagcggtacacatccaccaaggaggttctcgatgccaccctgattcaccagtccatcactggcctgtacgagacccgaatcgacctgtctcagcttggtggcgactccagagccgatcccaagaaaaagcgaaaggtctaagcggccgcaagtgtggatggggaagtgagtgcccggttctgtgtgcacaattggcaatccaagatggatggattcaacacagggatatagcgagctacgtggtggtgcgaggatatagcaacggatatttatgtttgacacttgagaatgtacgatacaagcactgtccaagtacaatactaaacatactgtacatactcatactcgtacccgggcaacggtttcacttgagtgcagtggctagtgctcttactcgtacagtgtgcaatactgcgtatcatagtctttgatgtatatcgtattcattcatgttagttgcgtacgagccggaagcataaagtgtaaagcctggggtgcctaatgagtgagctaactcacattaattgcgttgcgctcactgcccgctttccagtcgggaaacctgtcgtgccagctgcattaatgaatcggccaacgcgcggggagaggcggtttgcgtattgggcgctcttccgcttcctcgctcactgactcgctgcgctcggtcgttcggctgcggcgagcggtatcagctcactcaaaggcggtaatacggttatccacagaatcaggggataacgcaggaaagaacatgtgagcaaaaggccagcaaaaggccaggaaccgtaaaaaggccgcgttgctggcgtttttccataggctccgcccccctgacgagcatcacaaaaatcgacgctcaagtcagaggtggcgaaacccgacaggactataaagataccaggcgtttccccctggaagctccctcgtgcgctctcctgttccgaccctgccgcttaccggatacctgtccgcctttctcccttcgggaagcgtggcgctttctcatagctcacgctgtaggtatctcagttcggtgtaggtcgttcgctccaagctgggctgtgtgcacgaaccccccgttcagcccgaccgctgcgccttatccggtaactatcgtcttgagtccaacccggtaagacacgacttatcgccactggcagcagccactggtaacaggattagcagagcgaggtatgtaggcggtgctacagagttcttgaagtggtggcctaactacggctacactagaaggacagtatttggtatctgcgctctgctgaagccagttaccttcggaaaaagagttggtagctcttgatccggcaaacaaaccaccgctggtagcggtggtttttttgtttgcaagcagcagattacgcgcagaaaaaaaggatctcaagaagatcctttgatcttttctacggggtctgacgctcagtggaacgaaaactcacgttaagggattttggtcatgagattatcaaaaaggatcttcacctagatccttttaaattaaaaatgaagttttaaatcaatctaaagtatatatgagtaaacttggtctgacagttaccaatgcttaatcagtgaggcacctatctcagcgatctgtctatttcgttcatccatagttgcctgactccccgtcgtgtagataactacgatacgggagggcttaccatctggccccagtgctgcaatgataccgcgagacccacgctcaccggctccagatttatcagcaataaaccagccagccggaagggccgagcgcagaagtggtcctgcaactttatccgcctccatccagtctattaattgttgccgggaagctagagtaagtagttcgccagttaatagtttgcgcaacgttgttgccattgctacaggcatcgtggtgtcacgctcgtcgtttggtatggcttcattcagctccggttcccaacgatcaaggcgagttacatgatcccccatgttgtgcaaaaaagcggttagctccttcggtcctccgatcgttgtcagaagtaagttggccgcagtgttatcactcatggttatggcagcactgcataattctcttactgtcatgccatccgtaagatgcttttctgtgactggtgagtactcaaccaagtcattctgagaatagtgtatgcggcgaccgagttgctcttgcccggcgtcaatacgggataataccgcgccacatagcagaactttaaaagtgctcatcattggaaaacgttcttcggggcgaaaactctcaaggatcttaccgctgttgagatccagttcgatgtaacccactcgtgcacccaactgatcttcagcatcttttactttcaccagcgtttctgggtgagcaaaaacaggaaggcaaaatgccgcaaaaaagggaataagggcgacacggaaatgttgaatactcatactcttcctttttcaatattattgaagcatttatcagggttattgtctcatgagcggatacatatttgaatgtatttagaaaaataaacaaataggggttccgcgcacatttccccgaaaagtgccacctgacgcgccctgtagcggcgcattaagcgcggcgggtgtggtggttacgcgcagcgtgaccgctacacttgccagcgccctagcgcccgctcctttcgctttcttcccttcctttctcgccacgttcgccggctttccccgtcaagctctaaatcgggggctccctttagggttccgatttagtgctttacggcacctcgaccccaaaaaacttgattagggtgatggttcacgtagtgggccatcgccctgatagacggtttttcgccctttgacgttggagtccacgttctttaatagtggactcttgttccaaactggaacaacactcaaccctatctcggtctattcttttgatttataagggattttgccgatttcggcctattggttaaaaaatgagctgatttaacaaaaatttaacgcgaattttaacaaaatattaacgcttacaatttccattcgccattcaggctgcgcaactgttgggaagggcgatcggtgcgggcctcttcgctattacgccagctggcgaaagggggatgtgctgcaaggcgattaagttgggtaacgccagggttttcccagtcacgacgttgtaaaacgacggccagtgaattgtaatacgactcactatagggcgaattgggtaccgggccccccctcgaggtcgatggtgtcgataagcttgatatcgaattcatgtcacacaaaccgatcttcgcctcaaggaaacctaattctacatccgagagactgccgagatccagtctacactgattaattttcgggccaataatttaaaaaaatcgtgttatataatattatatgtattatatatatacatcatgatgatactgacagtcatgtcccattgctaaatagacagactccatctgccgcctccaactgatgttctcaatatttaaggggtcatctcgcattgtttaataataaacagactccatctaccgcctccaaatgatgttctcaaaatatattgtatgaacttatttttattacttagtattattagacaacttacttgctttatgaaaaacacttcctatttaggaaacaatttataatggcagttcgttcatttaacaatttatgtagaataaatgttataaatgcgtatgggaaatcttaaatatggatagcataaatgatatctgcattgcctaattcgaaatcaacagcaacgaaaaaaatcccttgtacaacataaatagtcatcgagaaatatcaactatcaaagaacagctattcacacgttactattgagattattattggacgagaatcacacactcaactgtctttctctcttctagaaatacaggtacaagtatgtactattctcattgttcatacttctagtcatttcatcccacatattccttggatttctctccaatgaatgacattctatcttgcaaattcaacaattataataagatataccaaagtagcggtatagtggcaatcaaaaagcttctctggtgtgcttctcgtatttatttttattctaatgatccattaaaggtatatatttatttcttgttatataatccttttgtttattacatgggctggatacataaaggtattttgatttaattttttgcttaaattcaatcccccctcgttcagtgtcaactgtaatggtaggaaattaccatacttttgaagaagcaaaaaaaatgaaagaaaaaaaaaatcgtatttccaggttagacgttccgcagaatctagaatgcggtatgcggtacattgttcttcgaacgtaaaagttgcgctccctgagatattgtacatttttgcttttacaagtacaagtacatcgtacaactatgtactactgttgatgcatccacaacagtttgttttgtttttttttgttttttttttttctaatgattcattaccgctatgtatacctacttgtacttgtagtaagccgggttattggcgttcaattaatcatagacttatgaatctgcacggtgtgcgctgcgagttacttttagcttatgcatgctacttgggtgtaatattgggatctgttcggaaatcaacggatgctcaat

SEQ ID NO: 55 - DNA, 1963 bp, synthetic construct
  misc_feature 1..1963: note = Hygromycin resistance cassette
  source 1..1963: mol_type = other DNA
gtttaaaccttaagcccgctcataacttcgtatagcatacattatacgaacggtaggttgcgggatagacgccgacggagggcaatggcgctatggaaccttgcggatatccatacgccgcggcggactgcgtccgaaccagctccagcagcgttttttccgggccattgagccgactgcgaccccgccaacgtgtcttggcccacgcactcatgtcatgttggtgttgggaggccactttttaagtagcacaaggcacctagctcgcagcaaggtgtccgaaccaaagaagcggctgcagtggtgcaaacggggcggaaacggcgggaaaaagccacgggggcacgaattgaggcacgccctcgaatttgagacgagtcacggccccattcgcccgcgcaatggctcgccaacgcccggtcttttgcaccacatcaggttaccccaagccaaacctttgtgttaaaaagcttaacatattataccgaacgtaggtttgggcgggcttgctccgtctgtccaaggcaacatttatataagggtctgcatcgccggctcaattgaatcttttttcttcttctcttctctatattcattcttgaattaaacacacatcaaccatggccaaaaagcctgaactcaccgcgacgtctgtcgagaagtttctgatcgaaaagttcgacagcgtctccgacctgatgcagctctcggagggcgaagaatctcgtgctttcagcttcgatgtaggagggcgtggatatgtcctgcgggtaaatagctgcgccgatggtttctacaaagatcgttatgtttatcggcactttgcatcggccgcgctcccgattccggaagtgcttgacattggggagttcagcgagagcctgacctattgcatctcccgccgtgcacagggtgtcacgttgcaagacctgcctgaaaccgaactgcccgctgttctgcagccggtcgcggaggctatggatgcgatcgctgcggccgatcttagccagacgagcgggttcggcccattcggaccgcaaggaatcggtcaatacactacatggcgtgatttcatatgcgcgattgctgatccccatgtgtatcactggcaaactgtgatggacgacaccgtcagtgcgtccgtcgcgcaggctctcgatgagctgatgctttgggccgaggactgccccgaagtccggcacctcgtgcacgcggatttcggctccaacaatgtcctgacggacaatggccgcataacagcggtcattgactggagcgaggcgatgttcggggattcccaatacgaggtcgccaacatcttcttctggaggccgtggttggcttgtatggagcagcagacgcgctacttcgagcggaggcatccggagcttgcaggatcgccgcggctccgggcgtatatgctccgcattggtcttgaccaactctatcagagcttggttgacggcaatttcgatgatgcagcttgggcgcagggtcgatgcgacgcaatcgtccgatccggagccgggactgtcgggcgtacacaaatcgcccgcagaagcgcggccgtctggaccgatggctgtgtagaagtactcgccgatagtggaaaccgacgccccagcactcgtccgagggcaaaggaatagcggccgcaagtgtggatggggaagtgagtgcccggttctgtgtgcacaattggcaatccaagatggatggattcaacacagggatatagcgagctacgtggtggtgcgaggatatagcaacggatatttatgtttgacacttgagaatgtacgatacaagcactgtccaagtacaatactaaacatactgtacatactcatactcgtacccgggcaacggtttcacttgagtgcagtggctagtgctcttactcgtacagtgtgctaccgttcgtatagcatacattatacgaagttatcatagtcttaattaa

SEQ ID NO: 56 - DNA, 1714 bp, Yarrowia lipolytica
  source 1..1714: mol_type = genomic DNA
catgacatgtgtccacagaccctcaatctggcctgatgagccaaatccatacgcgctttcgcagctctaaaggctataacaagtcacaccaccctgctcgacctcagcgccctcactttttgttaagacaaactgtacacgctgttccagcgttttctgcctgcacctggtgggacatttggtgcaacctaaagtgctcggaacctctgtggtgtccagatcagcgcagcagttccgaggtagttttgaggcccttagatgatggtttaaacgtcgacgagtatctgtctgactcgtcattgccgcctttggagtacgactccaactatgagtgtgcttggatcactttgacgatacattcttcgttggaggctgtgggtctgacagctgcgttttcggcgcggttggccgacaacaatatcagctgcaacgtcattgctggctttcatcatgatcacatttttgtcggcaaaggcgacgcccagagagccattgacgttctttctaatttggaccgatagccgtatagtccagtctatctataagttcaactaactcgtaactattaccataacatatacttcactgccccagataaggttccgataaaaagttctgcagactaaatttatttcagtctcctcttcaccaccaaaatgccctcctacgaagctcgagctaacgtccacaagtccgcctttgccgctcgagtgctcaagctcgtggcagccaagaaaaccaacctgtgtgcttctctggatgttaccaccaccaaggagctcattgagcttgccgataaggtcggaccttatgtgtgcatgatcaaaacccatatcgacatcattgacgacttcacctacgccggcactgtgctccccctcaaggaacttgctcttaagcacggtttcttcctgttcgaggacagaaagttcgcagatattggcaacactgtcaagcaccagtaccggtgtcaccgaatcgccgagtggtccgatatcaccaacgcccacggtgtacccggaaccggaatcattgctggcctgcgagctggtgccgaggaaactgtctctgaacagaagaaggaggacgtctctgactacgagaactcccagtacaaggagttcctagtcccctctcccaacgagaagctggccagaggtctgctcatgctggccgagctgtcttgcaagggctctctggccactggcgagtactccaagcagaccattgagcttgcccgatccgaccccgagtttgtggttggcttcattgcccagaaccgacctaagggcgactctgaggactggcttattctgacccccggggtgggtcttgacgacaagggagacgctctcggacagcagtaccgaactgttgaggatgtcatgtctaccggaacggatatcataattgtcggccgaggtctgtacggccagaaccgagatcctattgaggaggccaagcgataccagaaggctggctgggaggcttaccagaagattaactgttagaggttagactatggatatgtaatttaactgtgtatatagagagcgtgcaagtatggagcgcttgttcagcttgtatgatggtcagacgacctgtctgatcgagtatgtatgatactgcacaacctgtgtatccgcatgatctgtccaatggggcatgttgttgtgtttctcgatacggagatgctgggtacagtgctaatacg

SEQ ID NO: 57 - DNA, 23 bp, Yarrowia lipolytica
  misc_feature 1..23: note = ura3-1 target site
  source 1..23: mol_type = genomic DNA
cgctcgagtgctcaagctcgtgg

SEQ ID NO: 58 - DNA, 34 bp, synthetic construct
  misc_feature 1..34: note = ura3-1F
  source 1..34: mol_type = other DNA
aatgggacgccgctcgagtgctcaagctcggttt

SEQ ID NO: 59 - DNA, 34 bp, synthetic construct
  misc_feature 1..34: note = ura3-1R
  source 1..34: mol_type = other DNA
tctaaaaccgagcttgagcactcgagcggcgtcc

SEQ ID NO: 60 - DNA, 20 bp, synthetic construct
  misc_feature 1..20: note = DNA encoding Ura3-1 VT domain
  source 1..20: mol_type = other DNA
cgctcgagtgctcaagctcg

SEQ ID NO: 61 - DNA, 11631 bp, synthetic construct
  misc_feature 1..11631: note = pRF421
  source 1..11631: mol_type = other DNA
taagactatgataacttcgtataatgtatgctatacgaacggtagcacactgtacgagtaagagcactagccactgcactcaagtgaaaccgttgcccgggtacgagtatgagtatgtacagtatgtttagtattgtacttggacagtgcttgtatcgtacattctcaagtgtcaaacataaatatccgttgctatatcctcgcaccaccacgtagctcgctatatccctgtgttgaatccatccatcttggattgccaattgtgcacacagaaccgggcactcacttccccatccacacttgcggccgctattcctttgccctcggacgagtgctggggcgtcggtttccactatcggcgagtacttctacacagccatcggtccagacggccgcgcttctgcgggcgatttgtgtacgcccgacagtcccggctccggatcggacgattgcgtcgcatcgaccctgcgcccaagctgcatcatcgaaattgccgtcaaccaagctctgatagagttggtcaagaccaatgcggagcatatacgcccggagccgcggcgatcctgcaagctccggatgcctccgctcgaagtagcgcgtctgctgctccatacaagccaaccacggcctccagaagaagatgttggcgacctcgtattgggaatccccgaacatcgcctcgctccagtcaatgaccgctgttatgcggccattgtccgtcaggacattgttggagccgaaatccgcgtgcacgaggtgccggacttcggggcagtcctcggcccaaagcatcagctcatcgagagcctgcgcgacggacgcactgacggtgtcgtccatcacagtttgccagtgatacacatggggatcagcaatcgcgcatatgaaatcacgccatgtagtgtattgaccgattccttgcggtccgaatgggccgaacccgctcgtctggctaagatcggccgcagcgatcgcatccatagcctccgcgaccggctgcagaacagcgggcagttcggtttcaggcaggtcttgcaacgtgacaccctgtgcacggcgggagatgcaataggtcaggctctcgctgaactccccaatgtcaagcacttccggaatcgggagcgcggccgatgcaaagtgccgataaacataacgatctttgtagaaaccatcggcgcagctatttacccgcaggacatatccacgccctcctacatcgaagctgaaagcacgagattcttcgccctccgagagctgcatcaggtcggagacgctgtcgaacttttcgatcagaaacttctcgacagacgtcgcggtgagttcaggctttttggccatggttgatgtgtgtttaattcaagaatgaatatagagaagagaagaagaaaaaagattcaattgagccggcgatgcagacccttatataaatgttgccttggacagacggagcaagcccgcccaaacctacgttcggtataatatgttaagctttttaacacaaaggtttggcttggggtaacctgatgtggtgcaaaagaccgggcgttggcgagccattgcgcgggcgaatggggccgtgactcgtctcaaattcgagggcgtgcctcaattcgtgcccccgtggctttttcccgccgtttccgccccgtttgcaccactgcagccgcttctttggttcggacaccttgctgcgagctaggtgccttgtgctacttaaaaagtggcctcccaacaccaacatgacatgagtgcgtgggccaagacacgttggcggggtcgcagtcggctcaatggcccggaaaaaacgctgctggagctggttcggacgcagtccgccgcggcgtatggatatccgcaaggttccatagcgccattgccctccgtcggcgtctatcccgcaacctaccgttcgtataatgtatgctatacgaagttatgagcgggcttaaggtttaaaccatcatctaagggcctcaaaactacctcggaactgctgcgctgatctggacaccacagaggttccgagcactttaggttgcaccaaatgtcccaccaggtgcaggcagaaaacgctggaacagcgtgtacagtttgtcttaacaaaaagtgagggcgctgaggtcgagcagggtggtgtgacttgttatagcctttagagctgcgaaagcgcgtatggatttggctcatcaggccagattgagggtctgtggacacatgtcatgttagtgtacttcaatcgccccctggatatagccccgacaataggccgtggcctcatttttttgccttccgcacatttccattgctcggtacccacaccttgcttctcctgcacttgccaaccttaatactggtttacattgaccaacatcttacaagcggggggcttgtctagggtatatataaacagtggctctcccaatcggttgccagtctcttttttcctttctttccccacagattcgaaatctaaactacacatcacaccatggacaagaaatactccatcggcctggacattggaaccaactctgtcggctgggctgtcatcaccgacgagtacaaggtgccctccaagaaattcaaggtcctcggaaacaccgatcgacactccatcaagaaaaacctcattggtgccctgttgttcgattctggcgagactgccgaagctaccagactcaagcgaactgctcggcgacgttacacccgacggaagaaccgaatctgctacctgcaggagatcttttccaacgagatggccaaggtggacgattcgttctttcatcgactggaggaatccttcctcgtcgaggaagacaagaaacacgagcgtcatcccatctttggcaacattgtggacgaggttgcttaccacgagaagtatcctaccatctaccatctccgaaagaaactcgtcgattccaccgacaaggcggatctcagacttatctacctcgctctggcacacatgatcaagtttcgaggtcatttcctcatcgagggcgatctcaatcccgacaacagcgatgtggacaagctgttcattcagctcgttcagacctacaaccagctgttcgaggaaaaccccatcaatgcctccggagtcgatgcaaaggccatcttgtctgctcgactctcgaagagcagacgactggagaacctcattgcccaacttcctggcgagaaaaagaacggactgtttggcaacctcattgccctttctcttggtctcacacccaacttcaagtccaacttcgatctggcggaggacgccaagctccagctgtccaaggacacctacgacgatgacctcgacaacctgcttgcacagattggcgatcagtacgccgacctgtttctcgctgccaagaacctttcggatgctattctcttgtctgacattctgcgagtcaacaccgagatcacaaaggctcccctttctgcctccatgatcaagcgatacgacgagcaccatcaggatctcacactgctcaaggctcttgtccgacagcaactgcccgagaagtacaaggagatctttttcgatcagtcgaagaacggctacgctggatacatcgacggcggagcctctcaggaagagttctacaagttcatcaagccaattctcgagaagatggacggaaccgaggaactgcttgtcaagctcaatcgagaggatctgcttcggaagcaacgaaccttcgacaacggcagcattcctcatcagatccacctcggtgagctgcacgccattcttcgacgtcaggaagacttctacccctttctcaaggacaaccgagagaagatcgagaagattcttacctttcgaatcccctactatgttggtcctcttgccagaggaaactctcgatttgcttggatgactcgaaagtccgaggaaaccatcactccctggaacttcgaggaagtcgtggacaagggtgcctctgcacagtccttcatcgagcgaatgaccaacttcgacaagaatctgcccaacgagaaggttcttcccaagcattcgctgctctacgagtactttacagtctacaacgaactcaccaaagtcaagtacgttaccgagggaatgcgaaagcctgccttcttgtctggcgaacagaagaaagccattgtcgatctcctgttcaagaccaaccgaaaggtcactgttaagcagctcaaggaggactacttcaagaaaatcgagtgtttcgacagcgtcgagatttccggagttgaggaccgattcaacgcctctttgggcacctatcacgatctgctcaagattatcaaggacaaggattttctcgacaacgaggaaaacgaggacattctggaggacatcgtgctcactcttaccctgttcgaagatcgggagatgatcgaggaacgactcaagacatacgctcacctgttcgacgacaaggtcatgaaacaactcaagcgacgtagatacaccggctggggaagactttcgcgaaagctcatcaacggcatcagagacaagcagtccggaaagaccattctggactttctcaagtccgatggctttgccaaccgaaacttcatgcagctcattcacgacgattctcttaccttcaaggaggacatccagaaggcacaagtgtccggtcagggcgacagcttgcacgaacatattgccaacctggctggttcgccagccatcaagaaaggcattctccagactgtcaaggttgtcgacgagctggtgaaggtcatgggacgtcacaagcccgagaacattgtgatcgagatggccagagagaaccagacaactcaaaagggtcagaaaaactcgcgagagcggatgaagcgaatcgaggaaggcatcaaggagctgggatcccagattctcaaggagcatcccgtcgagaacactcaactgcagaacgagaagctgtatctctactatctgcagaatggtcgagacatgtacgtggatcaggaactggacatcaatcgtctcagcgactacgatgtggaccacattgtccctcaatcctttctcaaggacgattctatcgacaacaaggtccttacacgatccgacaagaacagaggcaagtcggacaacgttcccagcgaagaggtggtcaaaaagatgaagaactactggcgacagctgctcaacgccaagctcattacccagcgaaagttcgacaatcttaccaaggccgagcgaggcggtctgtccgagctcgacaaggctggcttcatcaagcgtcaactcgtcgagaccagacagatcacaaagcacgtcgcacagattctcgattctcggatgaacaccaagtacgacgagaacgacaagctcatccgagaggtcaaggtgattactctcaagtccaaactggtctccgatttccgaaaggactttcagttctacaaggtgcgagagatcaacaattaccaccatgcccacgatgcttacctcaacgccgtcgttggcactgcgctcatcaagaaataccccaagctcgaaagcgagttcgtttacggcgattacaaggtctacgacgttcgaaagatgattgccaagtccgaacaggagattggcaaggctactgccaagtacttcttttactccaacatcatgaactttttcaagaccgagatcaccttggccaacggagagattcgaaagagaccacttatcgagaccaacggcgaaactggagagatcgtgtgggacaagggtcgagactttgcaaccgtgcgaaaggttctgtcgatgcctcaggtcaacatcgtcaagaaaaccgaggttcagactggcggattctccaaggagtcgattctgcccaagcgaaactccgacaagctcatcgctcgaaagaaagactgggatcccaagaaatacggtggcttcgattctcctaccgtcgcctattccgtgcttgtcgttgcgaaggtcgagaagggcaagtccaaaaagctcaagtccgtcaaggagctgctcggaattaccatcatggagcgatcgagcttcgagaagaatcccatcgacttcttggaagccaagggttacaaggaggtcaagaaagacctcattatcaagctgcccaagtactctctgttcgaactggagaacggtcgaaagcgtatgctcgcctccgctggcgagctgcagaagggaaacgagcttgccttgccttcgaagtacgtcaactttctctatctggcttctcactacgagaagctcaagggttctcccgaggacaacgaacagaagcaactcttcgttgagcagcacaaacattacctcgacgagattatcgagcagatttccgagttttcgaagcgagtcatcctggctgatgccaacttggacaaggtgctctctgcctacaacaagcatcgggacaaacccattcgagaacaggcggagaacatcattcacctgtttactcttaccaacctgggtgctcctgcagctttcaagtacttcgataccactatcgaccgaaagcggtacacatccaccaaggaggttctcgatgccaccctgattcaccagtccatcactggcctgtacgagacccgaatcgacctgtctcagcttggtggcgactccagagccgatcccaagaaaaagcgaaaggtctaagcggccgcaagtgtggatggggaagtgagtgcccggttctgtgtgcacaattggcaatccaagatggatggattcaacacagggatatagcgagctacgtggtggtgcgaggatatagcaacggatatttatgtttgacacttgagaatgtacgatacaagcactgtccaagtacaatactaaacatactgtacatactcatactcgtacccgggcaacggtttcacttgagtgcagtggctagtgctcttactcgtacagtgtgcaatactgcgtatcatagtctttgatgtatatcgtattcattcatgttagttgcgtacgagccggaagcataaagtgtaaagcctggggtgcctaatgagtgagctaactcacattaattgcgttgcgctcactgcccgctttccagtcgggaaacctgtcgtgccagctgcattaatgaatcggccaacgcgcggggagaggcggtttgcgtattgggcgctcttccgcttcctcgctcactgactcgctgcgctcggtcgttcggctgcggcgagcggtatcagctcactcaaaggcggtaatacggttatccacagaatcaggggataacgcaggaaagaacatgtgagcaaaaggccagcaaaaggccaggaaccgtaaaaaggccgcgttgctggcgtttttccataggctccgcccccctgacgagcatcacaaaaatcgacgctcaagtcagaggtggcgaaacccgacaggactataaagataccaggcgtttccccctggaagctccctcgtgcgctctcctgttccgaccctgccgcttaccggatacctgtccgcctttctcccttcgggaagcgtggcgctttctcatagctcacgctgtaggtatctcagttcggtgtaggtcgttcgctccaagctgggctgtgtgcacgaaccccccgttcagcccgaccgctgcgccttatccggtaactatcgtcttgagtccaacccggtaagacacgacttatcgccactggcagcagccactggtaacaggattagcagagcgaggtatgtaggcggtgctacagagttcttgaagtggtggcctaactacggctacactagaaggacagtatttggtatctgcgctctgctgaagccagttaccttcggaaaaagagttggtagctcttgatccggcaaacaaaccaccgctggtagcggtggtttttttgtttgcaagcagcagattacgcgcagaaaaaaaggatctcaagaagatcctttgatcttttctacggggtctgacgctcagtggaacgaaaactcacgttaagggattttggtcatgagattatcaaaaaggatcttcacctagatccttttaaattaaaaatgaagttttaaatcaatctaaagtatatatgagtaaacttggtctgacagttaccaatgcttaatcagtgaggcacctatctcagcgatctgtctatttcgttcatccatagttgcctgactccccgtcgtgtagataactacgatacgggagggcttaccatctggccccagtgctgcaatgataccgcgagacccacgctcaccggctccagatttatcagcaataaaccagccagccggaagggccgagcgcagaagtggtcctgcaactttatccgcctccatccagtctattaattgttgccgggaagctagagtaagtagttcgccagttaatagtttgcgcaacgttgttgccattgctacaggcatcgtggtgtcacgctcgtcgtttggtatggcttcattcagctccggttcccaacgatcaaggcgagttacatgatcccccatgttgtgcaaaaaagcggttagctccttcggtcctccgatcgttgtcagaagtaagttggccgcagtgttatcactcatggttatggcagcactgcataattctcttactgtcatgccatccgtaagatgcttttctgtgactggtgagtactcaaccaagtcattctgagaatagtgtatgcggcgaccgagttgctcttgcccggcgtcaatacgggataataccgcgccacatagcagaactttaaaagtgctcatcattggaaaacgttcttcggggcgaaaactctcaaggatcttaccgctgttgagatccagttcgatgtaacccactcgtgcacccaactgatcttcagcatcttttactttcaccagcgtttctgggtgagcaaaaacaggaaggcaaaatgccgcaaaaaagggaataagggcgacacggaaatgttgaatactcatactcttcctttttcaatattattgaagcatttatcagggttattgtctcatgagcggatacatatttgaatgtatttagaaaaataaacaaataggggttccgcgcacatttccccgaaaagtgccacctgacgcgccctgtagcggcgcattaagcgcggcgggtgtggtggttacgcgcagcgtgaccgctacacttgccagcgccctagcgcccgctcctttcgctttcttcccttcctttctcgccacgttcgccggctttccccgtcaagctctaaatcgggggctccctttagggttccgatttagtgctttacggcacctcgaccccaaaaaacttgattagggtgatggttcacgtagtgggccatcgccctgatagacggtttttcgccctttgacgttggagtccacgttctttaatagtggactcttgttccaaactggaacaacactcaaccctatctcggtctattcttttgatttataagggattttgccgatttcggcctattggttaaaaaatgagctgatttaacaaaaatttaacgcgaattttaacaaaatattaacgcttacaatttccattcgccattcaggctgcgcaactgttgggaagggcgatcggtgcgggcctcttcgctattacgccagctggcgaaagggggatgtgctgcaaggcgattaagttgggtaacgccagggttttcccagtcacgacgttgtaaaacgacggccagtgaattgtaatacgactcactatagggcgaattgggtaccgggccccccctcgaggtcgatggtgtcgataagcttgatatcgaattcatgtcacacaaaccgatcttcgcctcaaggaaacctaattctacatccgagagactgccgagatccagtctacactgattaattttcgggccaataatttaaaaaaatcgtgttatataatattatatgtattatatatatacatcatgatgatactgacagtcatgtcccattgctaaatagacagactccatctgccgcctccaactgatgttctcaatatttaaggggtcatctcgcattgtttaataataaacagactccatctaccgcctccaaatgatgttctcaaaatatattgtatgaacttatttttattacttagtattattagacaacttacttgctttatgaaaaacacttcctatttaggaaacaatttataatggcagttcgttcatttaacaatttatgtagaataaatgttataaatgcgtatgggaaatcttaaatatggatagcataaatgatatctgcattgcctaattcgaaatcaacagcaacgaaaaaaatcccttgtacaacataaatagtcatcgagaaatatcaactatcaaagaacagctattcacacgttactattgagattattattggacgagaatcacacactcaactgtctttctctcttctagaaatacaggtacaagtatgtactattctcattgttcatacttctagtcatttcatcccacatattccttggatttctctccaatgaatgacattctatcttgcaaattcaacaattataataagatataccaaagtagcggtatagtggcaatcaaaaagcttctctggtgtgcttctcgtatttatttttattctaatgatccattaaaggtatatatttatttcttgttatataatccttttgtttattacatgggctggatacataaaggtattttgatttaattttttgcttaaattcaatcccccctcgttcagtgtcaactgtaatggtaggaaattaccatacttttgaagaagcaaaaaaaatgaaagaaaaaaaaaatcgtatttccaggttagacgttccgcagaatctagaatgcggtatgcggtacattgttcttcgaacgtaaaagttgcgctccctgagatattgtacatttttgcttttacaagtacaagtacatcgtacaactatgtactactgttgatgcatccacaacagtttgttttgtttttttttgttttttttttttctaatgattcattaccgctatgtatacctacttgtacttgtagtaagccgggttattggcgttcaattaatcatagacttatgaatctgcacggtgtgcgctgcgagttacttttagcttatgcatgctacttgggtgtaatattgggatctgttcggaaatcaacggatgctcaatcgataaaaaacaaaaaaaaaagcaccgactcggtgccactttttcaagttgataacggactagccttattttaacttgctatttctagctctaaaaccgagcttgagcactcgagcggcgtcccattcgccatgccgaagcatgttgcccagccggcgccagcgaggaggctgggaccatgccggccattattttgcgttaagtttctaatcatcacgaaattatctatcaaaaataactaggtcccaccgagattcgaactcgggaccttaagatttgcaatctcacgcgctaccgctgtgccataggaccgaagttaaaatttggccaaagaaggacctgggcaccctggactgtgggttagggtaatattccttatggagacaatgggctagggtaaattacctaaaatgggtcgataaagaggggtgttcccagttgggaagtgtaattgaagacggggtcaaaaaagaaaatcaaaaaaaatttaat

SEQ ID NO: 62 - DNA, 378 bp, Yarrowia lipolytica
  source 1..378: mol_type = genomic DNA
gagtatctgtctgactcgtcattgccgcctttggagtacgactccaactatgagtgtgcttggatcactttgacgatacattcttcgttggaggctgtgggtctgacagctgcgttttcggcgcggttggccgacaacaatatcagctgcaacgtcattgctggctttcatcatgatcacatttttgtcggcaaaggcgacgcccagagagccattgacgttctttctaatttggaccgatagccgtatagtccagtctatctataagttcaactaactcgtaactattaccataacatatacttcactgccccagataaggttccgataaaaagttctgcagactaaatttatttcagtctcctcttcaccaccaaa

SEQ ID NO: 63 - DNA, 258 bp, Yarrowia lipolytica
  source 1..258: mol_type = genomic DNA
tagaggttagactatggatatgtaatttaactgtgtatatagagagcgtgcaagtatggagcgcttgttcagcttgtatgatggtcagacgacctgtctgatcgagtatgtatgatactgcacaacctgtgtatccgcatgatctgtccaatggggcatgttgttgtgtttctcgatacggagatgctgggtacagtgctaatacgttgaactacttatacttatatgaggctcgaagaaagctgacttgtgtatgac

SEQ ID NO: 64 - DNA, 648 bp, synthetic construct
  misc_feature 1..648: note = URA3 deletion polynucleotide editing template
  source 1..648: mol_type = other DNA
gaattcgagtatctgtctgactcgtcattgccgcctttggagtacgactccaactatgagtgtgcttggatcactttgacgatacattcttcgttggaggctgtgggtctgacagctgcgttttcggcgcggttggccgacaacaatatcagctgcaacgtcattgctggctttcatcatgatcacatttttgtcggcaaaggcgacgcccagagagccattgacgttctttctaatttggaccgatagccgtatagtccagtctatctataagttcaactaactcgtaactattaccataacatatacttcactgccccagataaggttccgataaaaagttctgcagactaaatttatttcagtctcctcttcaccaccaaatagaggttagactatggatatgtaatttaactgtgtatatagagagcgtgcaagtatggagcgcttgttcagcttgtatgatggtcagacgacctgtctgatcgagtatgtatgatactgcacaacctgtgtatccgcatgatctgtccaatggggcatgttgttgtgtttctcgatacggagatgctgggtacagtgctaatacgttgaactacttatacttatatgaggctcgaagaaagctgacttgtgtatgacaagctt

SEQ ID NO: 65 - DNA, 3277 bp, synthetic construct
  misc_feature 1..3277: note = pRF263
  source 1..3277: mol_type = other DNA
agcttgtcatacacaagtcagctttcttcgagcctcatataagtataagtagttcaacgtattagcactgtacccagcatctccgtatcgagaaacacaacaacatgccccattggacagatcatgcggatacacaggttgtgcagtatcatacatactcgatcagacaggtcgtctgaccatcatacaagctgaacaagcgctccatacttgcacgctctctatatacacagttaaattacatatccatagtctaacctctatttggtggtgaagaggagactgaaataaatttagtctgcagaactttttatcggaaccttatctggggcagtgaagtatatgttatggtaatagttacgagttagttgaacttatagatagactggactatacggctatcggtccaaattagaaagaacgtcaatggctctctgggcgtcgcctttgccgacaaaaatgtgatcatgatgaaagccagcaatgacgttgcagctgatattgttgtcggccaaccgcgccgaaaacgcagctgtcagacccacagcctccaacgaagaatgtatcgtcaaagtgatccaagcacactcatagttggagtcgtactccaaaggcggcaatgacgagtcagacagatactcgaattcgtaatcatggtcatagctgtttcctgtgtgaaattgttatccgctcacaattccacacaacatacgagccggaagcataaagtgtaaagcctggggtgcctaatgagtgagctaactcacattaattgcgttgcgctcactgcccgctttccagtcgggaaacctgtcgtgccagctgcattaatgaatcggccaacgcgcggggagaggcggtttgcgtattgggcgctcttccgcttcctcgctcactgactcgctgcgctcggtcgttcggctgcggcgagcggtatcagctcactcaaaggcggtaatacggttatccacagaatcaggggataacgcaggaaagaacatgtgagcaaaaggccagcaaaaggccaggaaccgtaaaaaggccgcgttgctggcgtttttccataggctccgcccccctgacgagcatcacaaaaatcgacgctcaagtcagaggtggcgaaacccgacaggactataaagataccaggcgtttccccctggaagctccctcgtgcgctctcctgttccgaccctgccgcttaccggatacctgtccgcctttctcccttcgggaagcgtggcgctttctcatagctcacgctgtaggtatctcagttcggtgtaggtcgttcgctccaagctgggctgtgtgcacgaaccccccgttcagcccgaccgctgcgccttatccggtaactatcgtcttgagtccaacccggtaagacacgacttatcgccactggcagcagccactggtaacaggattagcagagcgaggtatgtaggcggtgctacagagttcttgaagtggtggcctaactacggctacactagaaggacagtatttggtatctgcgctctgctgaagccagttaccttcggaaaaagagttggtagctcttgatccggcaaacaaaccaccgctggtagcggtggtttttttgtttgcaagcagcagattacgcgcagaaaaaaaggatctcaagaagatcctttgatcttttctacggggtctgacgctcagtggaacgaaaactcacgttaagggattttggtcatgagattatcaaaaaggatcttcacctagatccttttaaattaaaaatgaagttttaaatcaatctaaagtatatatgagtaaacttggtctgacagttaccaatgcttaatcagtgaggcacctatctcagcgatctgtctatttcgttcatccatagttgcctgactccccgtcgtgtagataactacgatacgggagggcttaccatctggccccagtgctgcaatgataccgcgagacccacgctcaccggctccagatttatcagcaataaaccagccagccggaagggccgagcgcagaagtggtcctgcaactttatccgcctccatccagtctattaattgttgccgggaagctagagtaagtagttcgccagttaatagtttgcgcaacgttgttgccattgctacaggcatcgtggtgtcacgctcgtcgtttggtatggcttcattcagctccggttcccaacgatcaaggcgagttacatgatcccccatgttgtgcaaaaaagcggttagctccttcggtcctccgatcgttgtcagaagtaagttggccgcagtgttatcactcatggttatggcagcactgcataattctcttactgtcatgccatccgtaagatgcttttctgtgactggtgagtactcaaccaagtcattctgagaatagtgtatgcggcgaccgagttgctcttgcccggcgtcaatacgggataataccgcgccacatagcagaactttaaaagtgctcatcattggaaaacgttcttcggggcgaaaactctcaaggatcttaccgctgttgagatccagttcgatgtaacccactcgtgcacccaactgatcttcagcatcttttactttcaccagcgtttctgggtgagcaaaaacaggaaggcaaaatgccgcaaaaaagggaataagggcgacacggaaatgttgaatactcatactcttcctttttcaatattattgaagcatttatcagggttattgtctcatgagcggatacatatttgaatgtatttagaaaaataaacaaataggggttccgcgcacatttccccgaaaagtgccacctgacgtctaagaaaccattattatcatgacattaacctataaaaataggcgtatcacgaggccctttcgtctcgcgcgtttcggtgatgacggtgaaaacctctgacacatgcagctcccggagacggtcacagcttgtctgtaagcggatgccgggagcagacaagcccgtcagggcgcgtcagcgggtgttggcgggtgtcggggctggcttaactatgcggcatcagagcagattgtactgagagtgcaccatatgcggtgtgaaataccgcacagatgcgtaaggagaaaataccgcatcaggcgccattcgccattcaggctgcgcaactgttgggaagggcgatcggtgcgggcctcttcgctattacgccagctggcgaaagggggatgtgctgcaaggcgattaagttgggtaacgccagggttttcccagtcacgacgttgtaaaacgacggccagtgcca

SEQ ID NO: 66 - DNA, 26 bp, synthetic construct
  misc_feature 1..26: note = HY007
  source 1..26: mol_type = other DNA
cgggcagtgagcgcaacgcaattaat

SEQ ID NO: 67 - DNA, 29 bp, synthetic construct
  misc_feature 1..29: note = oligo 297
  source 1..29: mol_type = other DNA
ggggaattctgcaaggcgattaagttggg

SEQ ID NO: 68 - DNA, 873 bp, synthetic construct
  misc_feature 1..873: note = EcoRI flanked URA3 deletion template
  source 1..873: mol_type = other DNA
cgggcagtgagcgcaacgcaattaatgtgagttagctcactcattaggcaccccaggctttacactttatgcttccggctcgtatgttgtgtggaattgtgagcggataacaatttcacacaggaaacagctatgaccatgattacgaattcgagtatctgtctgactcgtcattgccgcctttggagtacgactccaactatgagtgtgcttggatcactttgacgatacattcttcgttggaggctgtgggtctgacagctgcgttttcggcgcggttggccgacaacaatatcagctgcaacgtcattgctggctttcatcatgatcacatttttgtcggcaaaggcgacgcccagagagccattgacgttctttctaatttggaccgatagccgtatagtccagtctatctataagttcaactaactcgtaactattaccataacatatacttcactgccccagataaggttccgataaaaagttctgcagactaaatttatttcagtctcctcttcaccaccaaatagaggttagactatggatatgtaatttaactgtgtatatagagagcgtgcaagtatggagcgcttgttcagcttgtatgatggtcagacgacctgtctgatcgagtatgtatgatactgcacaacctgtgtatccgcatgatctgtccaatggggcatgttgttgtgtttctcgatacggagatgctgggtacagtgctaatacgttgaactacttatacttatatgaggctcgaagaaagctgacttgtgtatgacaagcttggcactggccgtcgttttacaacgtcgtgactgggaaaaccctggcgttacccaacttaatcgccttgcagaattcccc

SEQ ID NO: 69 - DNA, 12349 bp, synthetic construct
  misc_feature 1..12349: note = pRF437
  source 1..12349: mol_type = other DNA
aattctgcaaggcgattaagttgggtaacgccagggttttcccagtcacgacgttgtaaaacgacggccagtgccaagcttgtcatacacaagtcagctttcttcgagcctcatataagtataagtagttcaacgtattagcactgtacccagcatctccgtatcgagaaacacaacaacatgccccattggacagatcatgcggatacacaggttgtgcagtatcatacatactcgatcagacaggtcgtctgaccatcatacaagctgaacaagcgctccatacttgcacgctctctatatacacagttaaattacatatccatagtctaacctctatttggtggtgaagaggagactgaaataaatttagtctgcagaactttttatcggaaccttatctggggcagtgaagtatatgttatggtaatagttacgagttagttgaacttatagatagactggactatacggctatcggtccaaattagaaagaacgtcaatggctctctgggcgtcgcctttgccgacaaaaatgtgatcatgatgaaagccagcaatgacgttgcagctgatattgttgtcggccaaccgcgccgaaaacgcagctgtcagacccacagcctccaacgaagaatgtatcgtcaaagtgatccaagcacactcatagttggagtcgtactccaaaggcggcaatgacgagtcagacagatactcgaattcatgtcacacaaaccgatcttcgcctcaaggaaacctaattctacatccgagagactgccgagatccagtctacactgattaattttcgggccaataatttaaaaaaatcgtgttatataatattatatgtattatatatatacatcatgatgatactgacagtcatgtcccattgctaaatagacagactccatctgccgcctccaactgatgttctcaatatttaaggggtcatctcgcattgtttaataataaacagactccatctaccgcctccaaatgatgttctcaaaatatattgtatgaacttatttttattacttagtattattagacaacttacttgctttatgaaaaacacttcctatttaggaaacaatttataatggcagttcgttcatttaacaatttatgtagaataaatgttataaatgcgtatgggaaatcttaaatatggatagcataaatgatatctgcattgcctaattcgaaatcaacagcaacgaaaaaaatcccttgtacaacataaatagtcatcgagaaatatcaactatcaaagaacagctattcacacgttactattgagattattattggacgagaatcacacactcaactgtctttctctcttctagaaatacaggtacaagtatgtactattctcattgttcatacttctagtcatttcatcccacatattccttggatttctctccaatgaatgacattctatcttgcaaattcaacaattataataagatataccaaagtagcggtatagtggcaatcaaaaagcttctctggtgtgcttctcgtatttatttttattctaatgatccattaaaggtatatatttatttcttgttatataatccttttgtttattacatgggctggatacataaaggtattttgatttaattttttgcttaaattcaatcccccctcgttcagtgtcaactgtaatggtaggaaattaccatacttttgaagaagcaaaaaaaatgaaagaaaaaaaaaatcgtatttccaggttagacgttccgcagaatctagaatgcggtatgcggtacattgttcttcgaacgtaaaagttgcgctccctgagatattgtacatttttgcttttacaagtacaagtacatcgtacaactatgtactactgttgatgcatccacaacagtttgttttgtttttttttgttttttttttttctaatgattcattaccgctatgtatacctacttgtacttgtagtaagccgggttattggcgttcaattaatcatagacttatgaatctgcacggtgtgcgctgcgagttacttttagcttatgcatgctacttgggtgtaatattgggatctgttcggaaatcaacggatgctcaatcgataaaaaacaaaaaaaaaagcaccgactcggtgccactttttcaagttgataacggactagccttattttaacttgctatttctagctctaaaaccgagcttgagcactcgagcggcgtcccattcgccatgccgaagcatgttgcccagccggcgccagcgaggaggctgggaccatgccggccattattttgcgttaagtttctaatcatcacgaaattatctatcaaaaataactaggtcccaccgagattcgaactcgggaccttaagatttgcaatctcacgcgctaccgctgtgccataggaccgaagttaaaatttggccaaagaaggacctgggcaccctggactgtgggttagggtaatattccttatggagacaatgggctagggtaaattacctaaaatgggtcgataaagaggggtgttcccagttgggaagtgtaattgaagacggggtcaaaaaagaaaatcaaaaaaaatttaattaagactatgataacttcgtataatgtatgctatacgaacggtagcacactgtacgagtaagagcactagccactgcactcaagtgaaaccgttgcccgggtacgagtatgagtatgtacagtatgtttagtattgtacttggacagtgcttgtatcgtacattctcaagtgtcaaacataaatatccgttgctatatcctcgcaccaccacgtagctcgctatatccctgtgttgaatccatccatcttggattgccaattgtgcacacagaaccgggcactcacttccccatccacacttgcggccgctattcctttgccctcggacgagtgctggggcgtcggtttccactatcggcgagtacttctacacagccatcggtccagacggccgcgcttctgcgggcgatttgtgtacgcccgacagtcccggctccggatcggacgattgcgtcgcatcgaccctgcgcccaagctgcatcatcgaaattgccgtcaaccaagctctgatagagttggtcaagaccaatgcggagcatatacgcccggagccgcggcgatcctgcaagctccggatgcctccgctcgaagtagcgcgtctgctgctccatacaagccaaccacggcctccagaagaagatgttggcgacctcgtattgggaatccccgaacatcgcctcgctccagtcaatgaccgctgttatgcggccattgtccgtcaggacattgttggagccgaaatccgcgtgcacgaggtgccggacttcggggcagtcctcggcccaaagcatcagctcatcgagagcctgcgcgacggacgcactgacggtgtcgtccatcacagtttgccagtgatacacatggggatcagcaatcgcgcatatgaaatcacgccatgtagtgtattgaccgattccttgcggtccgaatgggccgaacccgctcgtctggctaagatcggccgcagcgatcgcatccatagcctccgcgaccggctgcagaacagcgggcagttcggtttcaggcaggtcttgcaacgtgacaccctgtgcacggcgggagatgcaataggtcaggctctcgctgaactccccaatgtcaagcacttccggaatcgggagcgcggccgatgcaaagtgccgataaacataacgatctttgtagaaaccatcggcgcagctatttacccgcaggacatatccacgccctcctacatcgaagctgaaagcacgagattcttcgccctccgagagctgcatcaggtcggagacgctgtcgaacttttcgatcagaaacttctcgacagacgtcgcggtgagttcaggctttttggccatggttgatgtgtgtttaattcaagaatgaatatagagaagagaagaagaaaaaagattcaattgagccggcgatgcagacccttatataaatgttgccttggacagacggagcaagcccgcccaaacctacgttcggtataatatgttaagctttttaacacaaaggtttggcttggggtaacctgatgtggtgcaaaagaccgggcgttggcgagccattgcgcgggcgaatggggccgtgactcgtctcaaattcgagggcgtgcctcaattcgtgcccccgtggctttttcccgccgtttccgccccgtttgcaccactgcagccgcttctttggttcggacaccttgctgcgagctaggtgccttgtgctacttaaaaagtggcctcccaacaccaacatgacatgagtgcgtgggccaagacacgttggcggggtcgcagtcggctcaatggcccggaaaaaacgctgctggagctggttcggacgcagtccgccgcggcgtatggatatccgcaaggttccatagcgccattgccctccgtcggcgtctatcccgcaacctaccgttcgtataatgtatgctatacgaagttatgagcgggcttaaggtttaaaccatcatctaagggcctcaaaactacctcggaactgctgcgctgatctggacaccacagaggttccgagcactttaggttgcaccaaatgtcccaccaggtgcaggcagaaaacgctggaacagcgtgtacagtttgtcttaacaaaaagtgagggcgctgaggtcgagcagggtggtgtgacttgttatagcctttagagctgcgaaagcgcgtatggatttggctcatcaggccagattgagggtctgtggacacatgtcatgttagtgtacttcaatcgccccctggatatagccccgacaataggccgtggcctcatttttttgccttccgcacatttccattgctcggtacccacaccttgcttctcctgcacttgccaaccttaatactggtttacattgaccaacatcttacaagcggggggcttgtctagggtatatataaacagtggctctcccaatcggttgccagtctcttttttcctttctttccccacagattcgaaatctaaactacacatcacaccatggacaagaaatactccatcggcctggacattggaaccaactctgtcggctgggctgtcatcaccgacgagtacaaggtgccctccaagaaattcaaggtcctcggaaacaccgatcgacactccatcaagaaaaacctcattggtgccctgttgttcgattctggcgagactgccgaagctaccagactcaagcgaactgctcggcgacgttacacccgacggaagaaccgaatctgctacctgcaggagatcttttccaacgagatggccaaggtggacgattcgttctttcatcgactggaggaatccttcctcgtcgaggaagacaagaaacacgagcgtcatcccatctttggcaacattgtggacgaggttgcttaccacgagaagtatcctaccatctaccatctccgaaagaaactcgtcgattccaccgacaaggcggatctcagacttatctacctcgctctggcacacatgatcaagtttcgaggtcatttcctcatcgagggcgatctcaatcccgacaacagcgatgtggacaagctgttcattcagctcgttcagacctacaaccagctgttcgaggaaaaccccatcaatgcctccggagtcgatgcaaaggccatcttgtctgctcgactctcgaagagcagacgactggagaacctcattgcccaacttcctggcgagaaaaagaacggactgtttggcaacctcattgccctttctcttggtctcacacccaacttcaagtccaacttcgatctggcggaggacgccaagctccagctgtccaaggacacctacgacgatgacctcgacaacctgcttgcacagattggcgatcagtacgccgacctgtttctcgctgccaagaacctttcggatgctattctcttgtctgacattctgcgagtcaacaccgagatcacaaaggctcccctttctgcctccatgatcaagcgatacgacgagcaccatcaggatctcacactgctcaaggctcttgtccgacagcaactgcccgagaagtacaaggagatctttttcgatcagtcgaagaacggctacgctggatacatcgacggcggagcctctcaggaagagttctacaagttcatcaagccaattctcgagaagatggacggaaccgaggaactgcttgtcaagctcaatcgagaggatctgcttcggaagcaacgaaccttcgacaacggcagcattcctcatcagatccacctcggtgagctgcacgccattcttcgacgtcaggaagacttctacccctttctcaaggacaaccgagagaagatcgagaagattcttacctttcgaatcccctactatgttggtcctcttgccagaggaaactctcgatttgcttggatgactcgaaagtccgaggaaaccatcactccctggaacttcgaggaagtcgtggacaagggtgcctctgcacagtccttcatcgagcgaatgaccaacttcgacaagaatctgcccaacgagaaggttcttcccaagcattcgctgctctacgagtactttacagtctacaacgaactcaccaaagtcaagtacgttaccgagggaatgcgaaagcctgccttcttgtctggcgaacagaagaaagccattgtcgatctcctgttcaagaccaaccgaaaggtcactgttaagcagctcaaggaggactacttcaagaaaatcgagtgtttcgacagcgtcgagatttccggagttgaggaccgattcaacgcctctttgggcacctatcacgatctgctcaagattatcaaggacaaggattttctcgacaacgaggaaaacgaggacattctggaggacatcgtgctcactcttaccctgttcgaagatcgggagatgatcgaggaacgactcaagacatacgctcacctgttcgacgacaaggtcatgaaacaactcaagcgacgtagatacaccggctggggaagactttcgcgaaagctcatcaacggcatcagagacaagcagtccggaaagaccattctggactttctcaagtccgatggctttgccaaccgaaacttcatgcagctcattcacgacgattctcttaccttcaaggaggacatccagaaggcacaagtgtccggtcagggcgacagcttgcacgaacatattgccaacctggctggttcgccagccatcaagaaaggcattctccagactgtcaaggttgtcgacgagctggtgaaggtcatgggacgtcacaagcccgagaacattgtgatcgagatggccagagagaaccagacaactcaaaagggtcagaaaaactcgcgagagcggatgaagcgaatcgaggaaggcatcaaggagctgggatcccagattctcaaggagcatcccgtcgagaacactcaactgcagaacgagaagctgtatctctactatctgcagaatggtcgagacatgtacgtggatcaggaactggacatcaatcgtctcagcgactacgatgtggaccacattgtccctcaatcctttctcaaggacgattctatcgacaacaaggtccttacacgatccgacaagaacagaggcaagtcggacaacgttcccagcgaagaggtggtcaaaaagatgaagaactactggcgacagctgctcaacgccaagctcattacccagcgaaagttcgacaatcttaccaaggccgagcgaggcggtctgtccgagctcgacaaggctggcttcatcaagcgtcaactcgtcgagaccagacagatcacaaagcacgtcgcacagattctcgattctcggatgaacaccaagtacgacgagaacgacaagctcatccgagaggtcaaggtgattactctcaagtccaaactggtctccgatttccgaaaggactttcagttctacaaggtgcgagagatcaacaattaccaccatgcccacgatgcttacctcaacgccgtcgttggcactgcgctcatcaagaaataccccaagctcgaaagcgagttcgtttacggcgattacaaggtctacgacgttcgaaagatgattgccaagtccgaacaggagattggcaaggctactgccaagtacttcttttactccaacatcatgaactttttcaagaccgagatcaccttggccaacggagagattcgaaagagaccacttatcgagaccaacggcgaaactggagagatcgtgtgggacaagggtcgagactttgcaaccgtgcgaaaggttctgtcgatgcctcaggtcaacatcgtcaagaaaaccgaggttcagactggcggattctccaaggagtcgattctgcccaagcgaaactccgacaagctcatcgctcgaaagaaagactgggatcccaagaaatacggtggcttcgattctcctaccgtcgcctattccgtgcttgtcgttgcgaaggtcgagaagggcaagtccaaaaagctcaagtccgtcaaggagctgctcggaattaccatcatggagcgatcgagcttcgagaagaatcccatcgacttcttggaagccaagggttacaaggaggtcaagaaagacctcattatcaagctgcccaagtactctctgttcgaactggagaacggtcgaaagcgtatgctcgcctccgctggcgagctgcagaagggaaacgagcttgccttgccttcgaagtacgtcaactttctctatctggcttctcactacgagaagctcaagggttctcccgaggacaacgaacagaagcaactcttcgttgagcagcacaaacattacctcgacgagattatcgagcagatttccgagttttcgaagcgagtcatcctggctgatgccaacttggacaaggtgctctctgcctacaacaagcatcgggacaaacccattcgagaacaggcggagaacatcattcacctgtttactcttaccaacctgggtgctcctgcagctttcaagtacttcgataccactatcgaccgaaagcggtacacatccaccaaggaggttctcgatgccaccctgattcaccagtccatcactggcctgtacgagacccgaatcgacctgtctcagcttggtggcgactccagagccgatcccaagaaaaagcgaaaggtctaagcggccgcaagtgtggatggggaagtgagtgcccggttctgtgtgcacaattggcaatccaagatggatggattcaacacagggatatagcgagctacgtggtggtgcgaggatatagcaacggatatttatgtttgacacttgagaatgtacgatacaagcactgtccaagtacaatactaaacatactgtacatactcatactcgtacccgggcaacggtttcacttgagtgcagtggctagtgctcttactcgtacagtgtgcaatactgcgtatcatagtctttgatgtatatcgtattcattcatgttagttgcgtacgagccggaagcataaagtgtaaagcctggggtgcctaatgagtgagctaactcacattaattgcgttgcgctcactgcccgctttccagtcgggaaacctgtcgtgccagctgcattaatgaatcggccaacgcgcggggagaggcggtttgcgtattgggcgctcttccgcttcctcgctcactgactcgctgcgctcggtcgttcggctgcggcgagcggtatcagctcactcaaaggcggtaatacggttatccacagaatcaggggataacgcaggaaagaacatgtgagcaaaaggccagcaaaaggccaggaaccgtaaaaaggccgcgttgctggcgtttttccataggctccgcccccctgacgagcatcacaaaaatcgacgctcaagtcagaggtggcgaaacccgacaggactataaagataccaggcgtttccccctggaagctccctcgtgcgctctcctgttccgaccctgccgcttaccggatacctgtccgcctttctcccttcgggaagcgtggcgctttctcatagctcacgctgtaggtatctcagttcggtgtaggtcgttcgctccaagctgggctgtgtgcacgaaccccccgttcagcccgaccgctgcgccttatccggtaactatcgtcttgagtccaacccggtaagacacgacttatcgccactggcagcagccactggtaacaggattagcagagcgaggtatgtaggcggtgctacagagttcttgaagtggtggcctaactacggctacactagaaggacagtatttggtatctgcgctctgctgaagccagttaccttcggaaaaagagttggtagctcttgatccggcaaacaaaccaccgctggtagcggtggtttttttgtttgcaagcagcagattacgcgcagaaaaaaaggatctcaagaagatcctttgatcttttctacggggtctgacgctcagtggaacgaaaactcacgttaagggattttggtcatgagattatcaaaaaggatcttcacctagatccttttaaattaaaaatgaagttttaaatcaatctaaagtatatatgagtaaacttggtctgacagttaccaatgcttaatcagtgaggcacctatctcagcgatctgtctatttcgttcatccatagttgcctgactccccgtcgtgtagataactacgatacgggagggcttaccatctggccccagtgctgcaatgataccgcgagacccacgctcaccggctccagatttatcagcaataaaccagccagccggaagggccgagcgcagaagtggtcctgcaactttatccgcctccatccagtctattaattgttgccgggaagctagagtaagtagttcgccagttaatagtttgcgcaacgttgttgccattgctacaggcatcgtggtgtcacgctcgtcgtttggtatggcttcattcagctccggttcccaacgatcaaggcgagttacatgatcccccatgttgtgcaaaaaagcggttagctccttcggtcctccgatcgttgtcagaagtaagttggccgcagtgttatcactcatggttatggcagcactgcataattctcttactgtcatgccatccgtaagatgcttttctgtgactggtgagtactcaaccaagtcattctgagaatagtgtatgcggcgaccgagttgctcttgcccggcgtcaatacgggataataccgcgccacatagcagaactttaaaagtgctcatcattggaaaacgttcttcggggcgaaaactctcaaggatcttaccgctgttgagatccagttcgatgtaacccactcgtgcacccaactgatcttcagcatcttttactttcaccagcgtttctgggtgagcaaaaacaggaaggcaaaatgccgcaaaaaagggaataagggcgacacggaaatgttgaatactcatactcttcctttttcaatattattgaagcatttatcagggttattgtctcatgagcggatacatatttgaatgtatttagaaaaataaacaaataggggttccgcgcacatttccccgaaaagtgccacctgacgcgccctgtagcggcgcattaagcgcggcgggtgtggtggttacgcgcagcgtgaccgctacacttgccagcgccctagcgcccgctcctttcgctttcttcccttcctttctcgccacgttcgccggctttccccgtcaagctctaaatcgggggctccctttagggttccgatttagtgctttacggcacctcgaccccaaaaaacttgattagggtgatggttcacgtagtgggccatcgccctgatagacggtttttcgccctttgacgttggagtccacgttctttaatagtggactcttgttccaaactggaacaacactcaaccctatctcggtctattcttttgatttataagggattttgccgatttcggcctattggttaaaaaatgagctgatttaacaaaaatttaacgcgaattttaacaaaatattaacgcttacaatttccattcgccattcaggctgcgcaactgttgggaagggcgatcggtgcgggcctcttcgctattacgccagctggcgaaagggggatgtgctgcaaggcgattaagttgggtaacgccagggttttcccagtcacgacgttgtaaaacgacggccagtgaattgtaatacgactcactatagggcgaattgggtaccgggccccccctcgaggtcgatggtgtcgataagcttgatatcg

SEQ ID NO: 70 - DNA, 20 bp, synthetic construct
  misc_feature 1..20: note = oligo 308
  source 1..20: mol_type = other DNA
cgtattagcactgtacccag

SEQ ID NO: 71 - DNA, 20 bp, synthetic construct
  misc_feature 1..20: note = oligo 309
  source 1..20: mol_type = other DNA
catgacatgtgtccacagac

SEQ ID NO: 72 - DNA, 859 bp, synthetic construct
  misc_feature 1..859: note = URA3 locus deletion PCR product
  source 1..859: mol_type = other DNA
catgacatgtgtccacagaccctcaatctggcctgatgagccaaatccatacgcgctttcgcagctctaaaggctataacaagtcacaccaccctgctcgacctcagcgccctcactttttgttaagacaaactgtacacgctgttccagcgttttctgcctgcacctggtgggacatttggtgcaacctaaagtgctcggaacctctgtggtgtccagatcagcgcagcagttccgaggtagttttgaggcccttagatgatggtttaaacgtcgacgagtatctgtctgactcgtcattgccgcctttggagtacgactccaactatgagtgtgcttggatcactttgacgatacattcttcgttggaggctgtgggtctgacagctgcgttttcggcgcggttggccgacaacaatatcagctgcaacgtcattgctggctttcatcatgatcacatttttgtcggcaaaggcgacgcccagagagccattgacgttctttctaatttggaccgatagccgtatagtccagtctatctataagttcaactaactcgtaactattaccataacatatacttcactgccccagataaggttccgataaaaagttctgcagactaaatttatttcagtctcctcttcaccaccaaaaggttagactatggatatgtaatttaactgtgtatatagagagcgtgcaagtatggagcgcttgttcagcttgtatgatggtcagacgacctgtctgatcgagtatgtatgatactgcacaacctgtgtatccgcatgatctgtccaatggggcatgttgttgtgtttctcgatacggagatgctgggtacagtgctaatacg